European Patent Application EP 4 212 619 A1, published July 19, 2023. Title: METHOD FOR PERFORMING GENE EDITING ON TARGET SITE IN CELL. Applicant: BIORAY LABORATORIES INC. The sequence listing filed with the application follows.

SEQUENCE LISTING (44 sequences)

SEQ ID NO: 1 - DNA, 20 bp, Artificial Sequence
cgactggccagggcgcctgt

SEQ ID NO: 2 - DNA, 20 bp, Artificial Sequence
gggcggtgctacaactgggc

SEQ ID NO: 3 - DNA, 20 bp, Artificial Sequence
agagctagcacagactagag

SEQ ID NO: 4 - DNA, 20 bp, Artificial Sequence
acaaaactgtgctagacatg

SEQ ID NO: 5 - DNA, 20 bp, Artificial Sequence
agagcaacagtgctgtggcc

SEQ ID NO: 6 - DNA, 20 bp, Artificial Sequence
gagtagcgcgagcacagcta

SEQ ID NO: 7 - DNA, 20 bp, Artificial Sequence
ccggagaggacccagacacg

SEQ ID NO: 8 - DNA, 20 bp, Artificial Sequence
aaagcaagaggatggagagg

SEQ ID NO: 9 - DNA, 20 bp, Artificial Sequence
gagaggacccagacacgggg

SEQ ID NO: 10 - DNA, 20 bp, Artificial Sequence
agagtctctcagctggtaca

SEQ ID NO: 11 - DNA, 20 bp, Artificial Sequence
actcacgctggatagcctcc

SEQ ID NO: 12 - DNA, 3012 bp, Artificial Sequence
ccctgccaccgccccagcccccccgtcaggctgttgcaggcatcacacggtggaaagatctggaactgtggccatggtgtgaggccatccacaaggtggaagctttgagggggagccgattagccatggacagttgtcattcagtagggtcacctgtgccccagcgaagggggatgggccgggaaggcagaggccaggcacctgcccccagcaggggcagaggctgtgggcagccgggaggctcccagaggctccgacagaatgggagtggggttgagcccacccctcactgcagcccaggaacctgagcccagagggggccacccaccttccccaggcagggaggcccggcccccagggagatgggggggatgggggaggagaagggcctgcccccacccggcagcctcaggaggggcagctcgggcgggatatggaaagaggccacagcagtgagcagagacacagaggaggaaggggccctgagctggggagacccccacggggtagggcgtgggggccacgggcccacctcctccccatctcctctgtctccctgtctctgtctctctctccctcccccaccctctccccagtcctaccccctcctcacccctcctcccccagcactgcctctgtcactctcgcccacgtggatgtggaggaagagggggcgggagcaaggggcgggcaccctcccttcaacctgacctgggacagtttcccttccgctcacctccgcctgagcagtggagaaggcggcactctggtggggctgctccaggcatgcagatcccacataagatacattgatgagtttggacaaaccacaactagaatgcagtgaaaaaaatgctttatttgtgaaatttgtgatgctattgctttatttgtaaccattataagctgcaataaacaagttgtcgaggccgcggatccttcgaattctcacttgtacagctcgtccatgccgagagtgatcccggcggcggtcacgaactccagcaggaccatgtgatcgcgcttctcgttggggtctttgctcagcttggactgggtgctcaggtagtggttgtcgggcagcagcacggggccgtcgccgatgggggtgttctgctggtagtggtcggcgagctgcacgccgccgtcctcgatgttgtggcggatcttgaagttggccttgatgccgttcttctgcttgtcggcggtgatatagacgttgtcgctgaagtagttgtactccagcttgtgccccaggatgttgccgtcctccttgaagtcgatgcccttcagctcgatgcggttcaccagggtgtcgccctcgaacttcacctcggcgcgggtcttgtagttgccgtcgtccttgaagaagatggtgcgctcctggacgtagccttcgggcatggcggacttgaagaagtcgtgctgcttcatgtggtcggggtagcgggcgaagcactgcacgccccagctcagggtggtcacgagggtgggccagggcacgggcagcttgccggtggtgcagatgaacttcagggtcagcttgccgtaggtggcatcgccctcgccctcgccggacacgctgaacttgtggccgtttacgtcgccgtccagctcgaccaggatgggcaccaccccggtgaacagctcctcgcccttgctcaccatggtggctctagagtaggcgccggtcacagcttggatctgtaacggcgcagaacagaaaacgaaacaaagacgtagagttgagcaagcagggtcaggcaaagcgtggagagccggctgagtctaggtaggctccaagggagcgccggacaaaggcccggtctcgacctgagctttaaacttacctagacggcggacgcagttcaggaggcaccacaggcgggaggcggcagaacgcgactcaaccggcgtggatggcggcctcaggtagggcggcgggcgcgtgaaggagagatgcgagcccctcgaagcttcagctgtgttctggcggcaaacccgttgcgaaaaagaacgttcacggcgactactgcacttatatacggttctcccccaccctcgggaaaaaggcggagccagtacacgacatcactttcccagtttaccccgcgccaccttctctaggcacccgttcaattgccgacccctccccccaacttctcggggactgtgggcgatgtgcgctctgcccactgacgggcaccggagcggcgccctggccagtcgtctgggcggtgctacaactgggctggcggccaggatggttcttaggtaggtggggtcggcggtcaggtgtcccagagccaggggtctggagggaccttccaccctcagtccctggcaggtcggggggtgctgaggcgggcctggccctggcagcccaggggtcccggagcgaggggtctggagggacctttcactctcagtccctggcaggtcggggggtgctgtggcaggcccagccttggcccccagctctgccccttaccctgagctgtgtggctttgggcagctcgaactcctgggttcctctctgggccccaactcctcccctggcccaagtcccctctttgctcctgggcaggcaggacctctgtcccctctcagccggtccttggggctgcgtgtttctgtagaatgacgggtcaggctggccagaaccccaaaccttggccgtggggagtctgcgtggcggctctgccttgcccaggcatccttggtcctcactcgagttttcctaaggatgggatgagccccatgtgggactaaccttggctttacgacgtcaaagtttagatgagctggtgatatttttctcattatatccaaagtgtacctgttcgagtgaggacagttcttctgtctccaggatccctcctgggtggggattgtgcccgcctgggtctctgcccagattccagggctctccccgagccctgttcagaccatccgtgggggaggccttggcctcactctcccggatcgaggagagagggagcctcttcctgg

SEQ ID NO: 13 - DNA, 3012 bp, Artificial Sequence
aggcatcacacggtggaaagatctggaactgtggccatggtgtgaggccatccacaaggtggaagctttgagggggagccgattagccatggacagttgtcattcagtagggtcacctgtgccccagcgaagggggatgggccgggaaggcagaggccaggcacctgcccccagcaggggcagaggctgtgggcagccgggaggctcccagaggctccgacagaatgggagtggggttgagcccacccctcactgcagcccaggaacctgagcccagagggggccacccaccttccccaggcagggaggcccggcccccagggagatgggggggatgggggaggagaagggcctgcccccacccggcagcctcaggaggggcagctcgggcgggatatggaaagaggccacagcagtgagcagagacacagaggaggaaggggccctgagctggggagacccccacggggtagggcgtgggggccacgggcccacctcctccccatctcctctgtctccctgtctctgtctctctctccctcccccaccctctccccagtcctaccccctcctcacccctcctcccccagcactgcctctgtcactctcgcccacgtggatgtggaggaagagggggcgggagcaaggggcgggcaccctcccttcaacctgacctgggacagtttcccttccgctcacctccgcctgagcagtggagaaggcggcactctggtggggctgctccaggcatgcagatcccacaggcgccctggccagtcgtctgggcggtgctacaactgtaagatacattgatgagtttggacaaaccacaactagaatgcagtgaaaaaaatgctttatttgtgaaatttgtgatgctattgctttatttgtaaccattataagctgcaataaacaagttgtcgaggccgcggatccttcgaattctcacttgtacagctcgtccatgccgagagtgatcccggcggcggtcacgaactccagcaggaccatgtgatcgcgcttctcgttggggtctttgctcagcttggactgggtgctcaggtagtggttgtcgggcagcagcacggggccgtcgccgatgggggtgttctgctggtagtggtcggcgagctgcacgccgccgtcctcgatgttgtggcggatcttgaagttggccttgatgccgttcttctgcttgtcggcggtgatatagacgttgtcgctgaagtagttgtactccagcttgtgccccaggatgttgccgtcctccttgaagtcgatgcccttcagctcgatgcggttcaccagggtgtcgccctcgaacttcacctcggcgcgggtcttgtagttgccgtcgtccttgaagaagatggtgcgctcctggacgtagccttcgggcatggcggacttgaagaagtcgtgctgcttcatgtggtcggggtagcgggcgaagcactgcacgccccagctcagggtggtcacgagggtgggccagggcacgggcagcttgccggtggtgcagatgaacttcagggtcagcttgccgtaggtggcatcgccctcgccctcgccggacacgctgaacttgtggccgtttacgtcgccgtccagctcgaccaggatgggcaccaccccggtgaacagctcctcgcccttgctcaccatggtggctctagagtaggcgccggtcacagcttggatctgtaacggcgcagaacagaaaacgaaacaaagacgtagagttgagcaagcagggtcaggcaaagcgtggagagccggctgagtctaggtaggctccaagggagcgccggacaaaggcccggtctcgacctgagctttaaacttacctagacggcggacgcagttcaggaggcaccacaggcgggaggcggcagaacgcgactcaaccggcgtggatggcggcctcaggtagggcggcgggcgcgtgaaggagagatgcgagcccctcgaagcttcagctgtgttctggcggcaaacccgttgcgaaaaagaacgttcacggcgactactgcacttatatacggttctcccccaccctcgggaaaaaggcggagccagtacacgacatcactttcccagtttaccccgcgccaccttctctaggcacccgttcaattgccgacccctccccccaacttctcggggactgtgggcgatgtgcgctctgcccactgacgggcaccggagcggctggcggccaggatggttcttaggtaggtggggtcggcggtcaggtgtcccagagccaggggtctggagggaccttccaccctcagtccctggcaggtcggggggtgctgaggcgggcctggccctggcagcccaggggtcccggagcgaggggtctggagggacctttcactctcagtccctggcaggtcggggggtgctgtggcaggcccagccttggcccccagctctgccccttaccctgagctgtgtggctttgggcagctcgaactcctgggttcctctctgggccccaactcctcccctggcccaagtcccctctttgctcctgggcaggcaggacctctgtcccctctcagccggtccttggggctgcgtgtttctgtagaatgacgggtcaggctggccagaaccccaaaccttggccgtggggagtctgcgtggcggctctgccttgcccaggcatccttggtcctcactcgagttttcctaaggatgggatgagccccatgtgggactaaccttggctttacgacgtcaaagtttagatgagctggtgatatttttctcattatatccaaagtgtacctgttcgagtgaggacagttcttctgtctccaggatccctcctgggtggggattgtgcccgcctgggtctctgcccagattccagggctctccccgagccctgttcagaccatccgtgggggaggccttggcctcactctcccggatcgaggagagagggagcctcttcctgggctgcccgtgaccctgggccctctgtgtacactgtga

SEQ ID NO: 14 - DNA, 1812 bp, Artificial Sequence
accccctcctcacccctcctcccccagcactgcctctgtcactctcgcccacgtggatgtggaggaagagggggcgggagcaaggggcgggcaccctcccttcaacctgacctgggacagtttcccttccgctcacctccgcctgagcagtggagaaggcggcactctggtggggctgctccaggcatgcagatcccacataagatacattgatgagtttggacaaaccacaactagaatgcagtgaaaaaaatgctttatttgtgaaatttgtgatgctattgctttatttgtaaccattataagctgcaataaacaagttgtcgaggccgcggatccttcgaattctcacttgtacagctcgtccatgccgagagtgatcccggcggcggtcacgaactccagcaggaccatgtgatcgcgcttctcgttggggtctttgctcagcttggactgggtgctcaggtagtggttgtcgggcagcagcacggggccgtcgccgatgggggtgttctgctggtagtggtcggcgagctgcacgccgccgtcctcgatgttgtggcggatcttgaagttggccttgatgccgttcttctgcttgtcggcggtgatatagacgttgtcgctgaagtagttgtactccagcttgtgccccaggatgttgccgtcctccttgaagtcgatgcccttcagctcgatgcggttcaccagggtgtcgccctcgaacttcacctcggcgcgggtcttgtagttgccgtcgtccttgaagaagatggtgcgctcctggacgtagccttcgggcatggcggacttgaagaagtcgtgctgcttcatgtggtcggggtagcgggcgaagcactgcacgccccagctcagggtggtcacgagggtgggccagggcacgggcagcttgccggtggtgcagatgaacttcagggtcagcttgccgtaggtggcatcgccctcgccctcgccggacacgctgaacttgtggccgtttacgtcgccgtccagctcgaccaggatgggcaccaccccggtgaacagctcctcgcccttgctcaccatggtggctctagagtaggcgccggtcacagcttggatctgtaacggcgcagaacagaaaacgaaacaaagacgtagagttgagcaagcagggtcaggcaaagcgtggagagccggctgagtctaggtaggctccaagggagcgccggacaaaggcccggtctcgacctgagctttaaacttacctagacggcggacgcagttcaggaggcaccacaggcgggaggcggcagaacgcgactcaaccggcgtggatggcggcctcaggtagggcggcgggcgcgtgaaggagagatgcgagcccctcgaagcttcagctgtgttctggcggcaaacccgttgcgaaaaagaacgttcacggcgactactgcacttatatacggttctcccccaccctcgggaaaaaggcggagccagtacacgacatcactttcccagtttaccccgcgccaccttctctaggcacccgttcaattgccgacccctccccccaacttctcggggactgtgggcgatgtgcgctctgcccactgacgggcaccggagcggcgccctggccagtcgtctgggcggtgctacaactgggctggcggccaggatggttcttaggtaggtggggtcggcggtcaggtgtcccagagccaggggtctggagggaccttccaccctcagtccctggcaggtcggggggtgctgaggcgggcctggccctggcagcccaggggtcccggagcgaggggtctggag

SEQ ID NO: 15 - DNA, 2209 bp, Artificial Sequence
cagcctcaggaggggcagctcgggcgggatatggaaagaggccacagcagtgagcagagacacagaggaggaaggggccctgagctggggagacccccacggggtagggcgtgggggccacgggcccacctcctccccatctcctctgtctccctgtctctgtctctctctccctcccccaccctctccccagtcctaccccctcctcacccctcctcccccagcactgcctctgtcactctcgcccacgtggatgtggaggaagagggggcgggagcaaggggcgggcaccctcccttcaacctgacctgggacagtttcccttccgctcacctccgcctgagcagtggagaaggcggcactctggtggggctgctccaggcatgcagatcccacataagatacattgatgagtttggacaaaccacaactagaatgcagtgaaaaaaatgctttatttgtgaaatttgtgatgctattgctttatttgtaaccattataagctgcaataaacaagttgtcgaggccgcggatccttcgaattctcacttgtacagctcgtccatgccgagagtgatcccggcggcggtcacgaactccagcaggaccatgtgatcgcgcttctcgttggggtctttgctcagcttggactgggtgctcaggtagtggttgtcgggcagcagcacggggccgtcgccgatgggggtgttctgctggtagtggtcggcgagctgcacgccgccgtcctcgatgttgtggcggatcttgaagttggccttgatgccgttcttctgcttgtcggcggtgatatagacgttgtcgctgaagtagttgtactccagcttgtgccccaggatgttgccgtcctccttgaagtcgatgcccttcagctcgatgcggttcaccagggtgtcgccctcgaacttcacctcggcgcgggtcttgtagttgccgtcgtccttgaagaagatggtgcgctcctggacgtagccttcgggcatggcggacttgaagaagtcgtgctgcttcatgtggtcggggtagcgggcgaagcactgcacgccccagctcagggtggtcacgagggtgggccagggcacgggcagcttgccggtggtgcagatgaacttcagggtcagcttgccgtaggtggcatcgccctcgccctcgccggacacgctgaacttgtggccgtttacgtcgccgtccagctcgaccaggatgggcaccaccccggtgaacagctcctcgcccttgctcaccatggtggctctagagtaggcgccggtcacagcttggatctgtaacggcgcagaacagaaaacgaaacaaagacgtagagttgagcaagcagggtcaggcaaagcgtggagagccggctgagtctaggtaggctccaagggagcgccggacaaaggcccggtctcgacctgagctttaaacttacctagacggcggacgcagttcaggaggcaccacaggcgggaggcggcagaacgcgactcaaccggcgtggatggcggcctcaggtagggcggcgggcgcgtgaaggagagatgcgagcccctcgaagcttcagctgtgttctggcggcaaacccgttgcgaaaaagaacgttcacggcgactactgcacttatatacggttctcccccaccctcgggaaaaaggcggagccagtacacgacatcactttcccagtttaccccgcgccaccttctctaggcacccgttcaattgccgacccctccccccaacttctcggggactgtgggcgatgtgcgctctgcccactgacgggcaccggagcggcgccctggccagtcgtctgggcggtgctacaactgggctggcggccaggatggttcttaggtaggtggggtcggcggtcaggtgtcccagagccaggggtctggagggaccttccaccctcagtccctggcaggtcggggggtgctgaggcgggcctggccctggcagcccaggggtcccggagcgaggggtctggagggacctttcactctcagtccctggcaggtcggggggtgctgtggcaggcccagccttggcccccagctctgccccttaccctgagctgtgtggctttgggcagctcgaactcctgggttcctctctgggccccaactcctcccctggcccaagtcccctctttgctcctgggcaggcaggacctctgtcccctctcagcc

SEQ ID NO: 16 - DNA, 4612 bp, Artificial Sequence
ttcaacagaggttggaacaaggctctacagggctgggggcagagggaggttctgtccagaatctgccttcaggacaagtacagccagcaggggcagcttagccacttatccactgcctgggcgaggcacagggctatggaggcacctaccaaccaacagttctccagccccagagccccagcccctgaggcacaagggtgggtgtgccaggagacagttgctgcgggccaccttagctgtctggcagcacagtgggtgctgccaggctccctgggggccccccgccaagcccacctggccagctgggccccccccacctccccaccaagccacccacacagcctcacatctctgagacccgggagtggccctttgttcataaacgagagcttcctcgccgtggccgcgcctcgcagacatcatctttgatgctctttttccactgtttcggtgctttaatgttttcccttcagagccgggccgagtgtctctcggagccaggcagccgcgccagctgtcaggcggtttctagcctcgcttcggttattttaagctgatgagcctgacgcatctcatcactaatatcagcagtttcatttctcctgttttccattcgctgtaataaaatgctcagcacagaatacaaggagataagcaagccatttcacaaacgccgggccgccagccaggcccaggcactggaccccctgaaccaccccaccctggcacgagtgggctggagggcagggccccggggaagaaggtcaaggctggaaggggaggtcagcctcacagccagcccctgccaccgccccagcccccccgtcaggctgttgcaggcatcacacggtggaaagatctggaactgtggccatggtgtgaggccatccacaaggtggaagctttgagggggagccgattagccatggacagttgtcattcagtagggtcacctgtgccccagcgaagggggatgggccgggaaggcagaggccaggcacctgcccccagcaggggcagaggctgtgggcagccgggaggctcccagaggctccgacagaatgggagtggggttgagcccacccctcactgcagcccaggaacctgagcccagagggggccacccaccttccccaggcagggaggcccggcccccagggagatgggggggatgggggaggagaagggcctgcccccacccggcagcctcaggaggggcagctcgggcgggatatggaaagaggccacagcagtgagcagagacacagaggaggaaggggccctgagctggggagacccccacggggtagggcgtgggggccacgggcccacctcctccccatctcctctgtctccctgtctctgtctctctctccctcccccaccctctccccagtcctaccccctcctcacccctcctcccccagcactgcctctgtcactctcgcccacgtggatgtggaggaagagggggcgggagcaaggggcgggcaccctcccttcaacctgacctgggacagtttcccttccgctcacctccgcctgagcagtggagaaggcggcactctggtggggctgctccaggcatgcagatcccacataagatacattgatgagtttggacaaaccacaactagaatgcagtgaaaaaaatgctttatttgtgaaatttgtgatgctattgctttatttgtaaccattataagctgcaataaacaagttgtcgaggccgcggatccttcgaattctcacttgtacagctcgtccatgccgagagtgatcccggcggcggtcacgaactccagcaggaccatgtgatcgcgcttctcgttggggtctttgctcagcttggactgggtgctcaggtagtggttgtcgggcagcagcacggggccgtcgccgatgggggtgttctgctggtagtggtcggcgagctgcacgccgccgtcctcgatgttgtggcggatcttgaagttggccttgatgccgttcttctgcttgtcggcggtgatatagacgttgtcgctgaagtagttgtactccagcttgtgccccaggatgttgccgtcctccttgaagtcgatgcccttcagctcgatgcggttcaccagggtgtcgccctcgaacttcacctcggcgcgggtcttgtagttgccgtcgtccttgaagaagatggtgcgctcctggacgtagccttcgggcatggcggacttgaagaagtcgtgctgcttcatgtggtcggggtagcgggcgaagcactgcacgccccagctcagggtggtcacgagggtgggccagggcacgggcagcttgccggtggtgcagatgaacttcagggtcagcttgccgtaggtggcatcgccctcgccctcgccggacacgctgaacttgtggccgtttacgtcgccgtccagctcgaccaggatgggcaccaccccggtgaacagctcctcgcccttgctcaccatggtggctctagagtaggcgccggtcacagcttggatctgtaacggcgcagaacagaaaacgaaacaaagacgtagagttgagcaagcagggtcaggcaaagcgtggagagccggctgagtctaggtaggctccaagggagcgccggacaaaggcccggtctcgacctgagctttaaacttacctagacggcggacgcagttcaggaggcaccacaggcgggaggcggcagaacgcgactcaaccggcgtggatggcggcctcaggtagggcggcgggcgcgtgaaggagagatgcgagcccctcgaagcttcagctgtgttctggcggcaaacccgttgcgaaaaagaacgttcacggcgactactgcacttatatacggttctcccccaccctcgggaaaaaggcggagccagtacacgacatcactttcccagtttaccccgcgccaccttctctaggcacccgttcaattgccgacccctccccccaacttctcggggactgtgggcgatgtgcgctctgcccactgacgggcaccggagcggcgccctggccagtcgtctgggcggtgctacaactgggctggcggccaggatggttcttaggtaggtggggtcggcggtcaggtgtcccagagccaggggtctggagggaccttccaccctcagtccctggcaggtcggggggtgctgaggcgggcctggccctggcagcccaggggtcccggagcgaggggtctggagggacctttcactctcagtccctggcaggtcggggggtgctgtggcaggcccagccttggcccccagctctgccccttaccctgagctgtgtggctttgggcagctcgaactcctgggttcctctctgggccccaactcctcccctggcccaagtcccctctttgctcctgggcaggcaggacctctgtcccctctcagccggtccttggggctgcgtgtttctgtagaatgacgggtcaggctggccagaaccccaaaccttggccgtggggagtctgcgtggcggctctgccttgcccaggcatccttggtcctcactcgagttttcctaaggatgggatgagccccatgtgggactaaccttggctttacgacgtcaaagtttagatgagctggtgatatttttctcattatatccaaagtgtacctgttcgagtgaggacagttcttctgtctccaggatccctcctgggtggggattgtgcccgcctgggtctctgcccagattccagggctctccccgagccctgttcagaccatccgtgggggaggccttggcctcactctcccggatcgaggagagagggagcctcttcctgggctgcccgtgaccctgggccctctgtgtacactgtgaccacagcccgctcctggaccctctgtgcccggctggccctctgtgcccagccagcctgcacctggggatgccaaggcctggggagggtggtttcacccaggccaagcctaagacagtccctctgggccctgctgggtaccggggtgtgacaccactgggaggacaagatgaggggcacccctggggccgccctgacaccccctcgaggctcctgccccgggggtcctggtgccccttcactgtggcaggcgactgggggttccccacctcggcccctctcccggggcctgctccccggcacctgaggcagcatccttgtcagggccgtgccttcctgcctcagcgccacctcttaaggttggcccgtgggtcactcaggactcagaactggagattctgggcaaaaggcaaagagcaaagggccaaaaggcatcccagggagacgactgcgggggaaccagagggcagaggggcgctcgtcacaggggagggggagctgagcgaggcaggaggggagccgagcctctccccccgtgtcccggctcttcaggcacgccctcgggacgccaccctccccgacccaggcgggaaagataagagcaaggtgtccgcagcctgacactcgtgcctcaggtgcccgcgcttgtgccggacaagactctcacaggtggcatgcctcggtttccccactggtaacagcacagggcactcagcaaggcgcagtgggcatgactggggtcctgtgggtcctgacccagatgtg

SEQ ID NO: 17 - DNA, 1858 bp, Artificial Sequence
gtcactctcgcccacgtggatgtggaggaagagggggcgggagcaaggggcgggcaccctcccttcaacctgacctgggacagtttcccttccgctcacctccgcctgagcagtggagaaggcggcactctggtggggctgctccaggcatgcagatcccacaggcgccctggccagtcgtctgggcggtgctacaactgtaagatacattgatgagtttggacaaaccacaactagaatgcagtgaaaaaaatgctttatttgtgaaatttgtgatgctattgctttatttgtaaccattataagctgcaataaacaagttgtcgaggccgcggatccttcgaattctcacttgtacagctcgtccatgccgagagtgatcccggcggcggtcacgaactccagcaggaccatgtgatcgcgcttctcgttggggtctttgctcagcttggactgggtgctcaggtagtggttgtcgggcagcagcacggggccgtcgccgatgggggtgttctgctggtagtggtcggcgagctgcacgccgccgtcctcgatgttgtggcggatcttgaagttggccttgatgccgttcttctgcttgtcggcggtgatatagacgttgtcgctgaagtagttgtactccagcttgtgccccaggatgttgccgtcctccttgaagtcgatgcccttcagctcgatgcggttcaccagggtgtcgccctcgaacttcacctcggcgcgggtcttgtagttgccgtcgtccttgaagaagatggtgcgctcctggacgtagccttcgggcatggcggacttgaagaagtcgtgctgcttcatgtggtcggggtagcgggcgaagcactgcacgccccagctcagggtggtcacgagggtgggccagggcacgggcagcttgccggtggtgcagatgaacttcagggtcagcttgccgtaggtggcatcgccctcgccctcgccggacacgctgaacttgtggccgtttacgtcgccgtccagctcgaccaggatgggcaccaccccggtgaacagctcctcgcccttgctcaccatggtggctctagagtaggcgccggtcacagcttggatctgtaacggcgcagaacagaaaacgaaacaaagacgtagagttgagcaagcagggtcaggcaaagcgtggagagccggctgagtctaggtaggctccaagggagcgccggacaaaggcccggtctcgacctgagctttaaacttacctagacggcggacgcagttcaggaggcaccacaggcgggaggcggcagaacgcgactcaaccggcgtggatggcggcctcaggtagggcggcgggcgcgtgaaggagagatgcgagcccctcgaagcttcagctgtgttctggcggcaaacccgttgcgaaaaagaacgttcacggcgactactgcacttatatacggttctcccccaccctcgggaaaaaggcggagccagtacacgacatcactttcccagtttaccccgcgccaccttctctaggcacccgttcaattgccgacccctccccccaacttctcggggactgtgggcgatgtgcgctctgcccactgacgggcaccggagcggctggcggccaggatggttcttaggtaggtggggtcggcggtcaggtgtcccagagccaggggtctggagggaccttccaccctcagtccctggcaggtcggggggtgctgaggcgggcctggccctggcagcccaggggtcccggagcgaggggtctggagggacctttcactctcagtccctggcaggtcggggggtgctgtggcaggcccagccttggcccccagctctgccccttaccctg

SEQ ID NO: 18 - DNA, 2212 bp, Artificial Sequence
aaagaggccacagcagtgagcagagacacagaggaggaaggggccctgagctggggagacccccacggggtagggcgtgggggccacgggcccacctcctccccatctcctctgtctccctgtctctgtctctctctccctcccccaccctctccccagtcctaccccctcctcacccctcctcccccagcactgcctctgtcactctcgcccacgtggatgtggaggaagagggggcgggagcaaggggcgggcaccctcccttcaacctgacctgggacagtttcccttccgctcacctccgcctgagcagtggagaaggcggcactctggtggggctgctccaggcatgcagatcccacaggcgccctggccagtcgtctgggcggtgctacaactgtaagatacattgatgagtttggacaaaccacaactagaatgcagtgaaaaaaatgctttatttgtgaaatttgtgatgctattgctttatttgtaaccattataagctgcaataaacaagttgtcgaggccgcggatccttcgaattctcacttgtacagctcgtccatgccgagagtgatcccggcggcggtcacgaactccagcaggaccatgtgatcgcgcttctcgttggggtctttgctcagcttggactgggtgctcaggtagtggttgtcgggcagcagcacggggccgtcgccgatgggggtgttctgctggtagtggtcggcgagctgcacgccgccgtcctcgatgttgtggcggatcttgaagttggccttgatgccgttcttctgcttgtcggcggtgatatagacgttgtcgctgaagtagttgtactccagcttgtgccccaggatgttgccgtcctccttgaagtcgatgcccttcagctcgatgcggttcaccagggtgtcgccctcgaacttcacctcggcgcgggtcttgtagttgccgtcgtccttgaagaagatggtgcgctcctggacgtagccttcgggcatggcggacttgaagaagtcgtgctgcttcatgtggtcggggtagcgggcgaagcactgcacgccccagctcagggtggtcacgagggtgggccagggcacgggcagcttgccggtggtgcagatgaacttcagggtcagcttgccgtaggtggcatcgccctcgccctcgccggacacgctgaacttgtggccgtttacgtcgccgtccagctcgaccaggatgggcaccaccccggtgaacagctcctcgcccttgctcaccatggtggctctagagtaggcgccggtcacagcttggatctgtaacggcgcagaacagaaaacgaaacaaagacgtagagttgagcaagcagggtcaggcaaagcgtggagagccggctgagtctaggtaggctccaagggagcgccggacaaaggcccggtctcgacctgagctttaaacttacctagacggcggacgcagttcaggaggcaccacaggcgggaggcggcagaacgcgactcaaccggcgtggatggcggcctcaggtagggcggcgggcgcgtgaaggagagatgcgagcccctcgaagcttcagctgtgttctggcggcaaacccgttgcgaaaaagaacgttcacggcgactactgcacttatatacggttctcccccaccctcgggaaaaaggcggagccagtacacgacatcactttcccagtttaccccgcgccaccttctctaggcacccgttcaattgccgacccctccccccaacttctcggggactgtgggcgatgtgcgctctgcccactgacgggcaccggagcggctggcggccaggatggttcttaggtaggtggggtcggcggtcaggtgtcccagagccaggggtctggagggaccttccaccctcagtccctggcaggtcggggggtgctgaggcgggcctggccctggcagcccaggggtcccggagcgaggggtctggagggacctttcactctcagtccctggcaggtcggggggtgctgtggcaggcccagccttggcccccagctctgccccttaccctgagctgtgtggctttgggcagctcgaactcctgggttcctctctgggccccaactcctcccctggcccaagtcccctctttgctcctgggcaggcaggacctctgtcccctctcagccggtccttggggctgcgtgtttctgtagaatgacgggt

SEQ ID NO: 19 - DNA, 4611 bp, Artificial Sequence
gcagagggaggttctgtccagaatctgccttcaggacaagtacagccagcaggggcagcttagccacttatccactgcctgggcgaggcacagggctatggaggcacctaccaaccaacagttctccagccccagagccccagcccctgaggcacaagggtgggtgtgccaggagacagttgctgcgggccaccttagctgtctggcagcacagtgggtgctgccaggctccctgggggccccccgccaagcccacctggccagctgggccccccccacctccccaccaagccacccacacagcctcacatctctgagacccgggagtggccctttgttcataaacgagagcttcctcgccgtggccgcgcctcgcagacatcatctttgatgctctttttccactgtttcggtgctttaatgttttcccttcagagccgggccgagtgtctctcggagccaggcagccgcgccagctgtcaggcggtttctagcctcgcttcggttattttaagctgatgagcctgacgcatctcatcactaatatcagcagtttcatttctcctgttttccattcgctgtaataaaatgctcagcacagaatacaaggagataagcaagccatttcacaaacgccgggccgccagccaggcccaggcactggaccccctgaaccaccccaccctggcacgagtgggctggagggcagggccccggggaagaaggtcaaggctggaaggggaggtcagcctcacagccagcccctgccaccgccccagcccccccgtcaggctgttgcaggcatcacacggtggaaagatctggaactgtggccatggtgtgaggccatccacaaggtggaagctttgagggggagccgattagccatggacagttgtcattcagtagggtcacctgtgccccagcgaagggggatgggccgggaaggcagaggccaggcacctgcccccagcaggggcagaggctgtgggcagccgggaggctcccagaggctccgacagaatgggagtggggttgagcccacccctcactgcagcccaggaacctgagcccagagggggccacccaccttccccaggcagggaggcccggcccccagggagatgggggggatgggggaggagaagggcctgcccccacccggcagcctcaggaggggcagctcgggcgggatatggaaagaggccacagcagtgagcagagacacagaggaggaaggggccctgagctggggagacccccacggggtagggcgtgggggccacgggcccacctcctccccatctcctctgtctccctgtctctgtctctctctccctcccccaccctctccccagtcctaccccctcctcacccctcctcccccagcactgcctctgtcactctcgcccacgtggatgtggaggaagagggggcgggagcaaggggcgggcaccctcccttcaacctgacctgggacagtttcccttccgctcacctccgcctgagcagtggagaaggcggcactctggtggggctgctccaggcatgcagatcccacaggcgccctggccagtcgtctgggcggtgctacaactgtaagatacattgatgagtttggacaaaccacaactagaatgcagtgaaaaaaatgctttatttgtgaaatttgtgatgctattgctttatttgtaaccattataagctgcaataaacaagttgtcgaggccgcggatccttcgaattctcacttgtacagctcgtccatgccgagagtgatcccggcggcggtcacgaactccagcaggaccatgtgatcgcgcttctcgttggggtctttgctcagcttggactgggtgctcaggtagtggttgtcgggcagcagcacggggccgtcgccgatgggggtgttctgctggtagtggtcggcgagctgcacgccgccgtcctcgatgttgtggcggatcttgaagttggccttgatgccgttcttctgcttgtcggcggtgatatagacgttgtcgctgaagtagttgtactccagcttgtgccccaggatgttgccgtcctccttgaagtcgatgcccttcagctcgatgcggttcaccagggtgtcgccctcgaacttcacctcggcgcgggtcttgtagttgccgtcgtccttgaagaagatggtgcgctcctggacgtagccttcgggcatggcggacttgaagaagtcgtgctgcttcatgtggtcggggtagcgggcgaagcactgcacgccccagctcagggtggtcacgagggtgggccagggcacgggcagcttgccggtggtgcagatgaacttcagggtcagcttgccgtaggtggcatcgccctcgccctcgccggacacgctgaacttgtggccgtttacgtcgccgtccagctcgaccaggatgggcaccaccccggtgaacagctcctcgcccttgctcaccatggtggctctagagtaggcgccggtcacagcttggatctgtaacggcgcagaacagaaaacgaaacaaagacgtagagttgagcaagcagggtcaggcaaagcgtggagagccggctgagtctaggtaggctccaagggagcgccggacaaaggcccggtctcgacctgagctttaaacttacctagacggcggacgcagttcaggaggcaccacaggcgggaggcggcagaacgcgactcaaccggcgtggatggcggcctcaggtagggcggcgggcgcgtgaaggagagatgcgagcccctcgaagcttcagctgtgttctggcggcaaacccgttgcgaaaaagaacgttcacggcgactactgcacttatatacggttctcccccaccctcgggaaaaaggcggagccagtacacgacatcactttcccagtttaccccgcgccaccttctctaggcacccgttcaattgccgacccctccccccaacttctcggggactgtgggcgatgtgcgctctgcccactgacgggcaccggagcggctggcggccaggatggttcttaggtaggtggggtcggcggtcaggtgtcccagagccaggggtctggagggaccttccaccctcagtccctggcaggtcggggggtgctgaggcgggcctggccctggcagcccaggggtcccggagcgaggggtctggagggacctttcactctcagtccctggcaggtcggggggtgctgtggcaggcccagccttggcccccagctctgccccttaccctgagctgtgtggctttgggcagctcgaactcctgggttcctctctgggccccaactcctcccctggcccaagtcccctctttgctcctgggcaggcaggacctctgtcccctctcagccggtccttggggctgcgtgtttctgtagaatgacgggtcaggctggccagaaccccaaaccttggccgtggggagtctgcgtggcggctctgccttgcccaggcatccttggtcctcactcgagttttcctaaggatgggatgagccccatgtgggactaaccttggctttacgacgtcaaagtttagatgagctggtgatatttttctcattatatccaaagtgtacctgttcgagtgaggacagttcttctgtctccaggatccctcctgggtggggattgtgcccgcctgggtctctgcccagattccagggctctccccgagccctgttcagaccatccgtgggggaggccttggcctcactctcccggatcgaggagagagggagcctcttcctgggctgcccgtgaccctgggccctctgtgtacactgtgaccacagcccgctcctggaccctctgtgcccggctggccctctgtgcccagccagcctgcacctggggatgccaaggcctggggagggtggtttcacccaggccaagcctaagacagtccctctgggccctgctgggtaccggggtgtgacaccactgggaggacaagatgaggggcacccctggggccgccctgacaccccctcgaggctcctgccccgggggtcctggtgccccttcactgtggcaggcgactgggggttccccacctcggcccctctcccggggcctgctccccggcacctgaggcagcatccttgtcagggccgtgccttcctgcctcagcgccacctcttaaggttggcccgtgggtcactcaggactcagaactggagattctgggcaaaaggcaaagagcaaagggccaaaaggcatcccagggagacgactgcgggggaaccagagggcagaggggcgctcgtcacaggggagggggagctgagcgaggcaggaggggagccgagcctctccccccgtgtcccggctcttcaggcacgccctcgggacgccaccctccccgacccaggcgggaaagataagagcaaggtgtccgcagcctgacactcgtgcctcaggtgcccgcgcttgtgccggacaagactctcacaggtggcatgcctcggtttccccactggtaacagcacagggcactcagcaaggcgcagtgggcatgactggggtcctgtgggtcctgacccagatgtggccaccccggccgcagtggtcttcattccaggatgcc

SEQ ID NO: 20 - DNA, 3012 bp, Artificial Sequence
gatccgccccgtcgttcctggccctgggctttgccaccctatgctgacaccccgtcccagtcccccttaccattccccttcgaccaccccacttccgaattggagccgcttcaactggccctgggcttagccactctgtgctgaccactctgccccaggcctccttaccattccccttcgacctactctcttccgcattggagtcgctttaactggccctggctttggcagcctgtgctgacccatgcagtcctccttaccatccctccctcgacttcccctcttccgatgttgagcccctccagccggtcctggactttgtctccttccctgccctgccctctcctgaacctgagccagctcccatagctcagtctggtctatctgcctggccctggccattgtcactttgcgctgccctcctctcgcccccgagtgcccttgctgtgccgccggaactctgccctctaacgctgccgtctctctcctgagtccggaccactttgagctctactggcttctgcgccgcctctggcccactgtttccccttcccaggcaggtcctgctttctctgacctgcattctctcccctgggcctgtgccgctttctgtctgcagcttgtggcctgggtcacctctacggctggcccagatccttccctgccgcctccttcaggttccgtcttcctccactccctcttccccttgctctctgctgtgttgctgcccaaggatgctctttccggagcacttccttctcggcgctgcaccacgtgatgtcctctgagcggatcctccctaagatacattgatgagtttggacaaaccacaactagaatgcagtgaaaaaaatgctttatttgtgaaatttgtgatgctattgctttatttgtaaccattataagctgcaataaacaagttgtcgaggccgcggatccttcgaattctcacttgtacagctcgtccatgccgagagtgatcccggcggcggtcacgaactccagcaggaccatgtgatcgcgcttctcgttggggtctttgctcagcttggactgggtgctcaggtagtggttgtcgggcagcagcacggggccgtcgccgatgggggtgttctgctggtagtggtcggcgagctgcacgccgccgtcctcgatgttgtggcggatcttgaagttggccttgatgccgttcttctgcttgtcggcggtgatatagacgttgtcgctgaagtagttgtactccagcttgtgccccaggatgttgccgtcctccttgaagtcgatgcccttcagctcgatgcggttcaccagggtgtcgccctcgaacttcacctcggcgcgggtcttgtagttgccgtcgtccttgaagaagatggtgcgctcctggacgtagccttcgggcatggcggacttgaagaagtcgtgctgcttcatgtggtcggggtagcgggcgaagcactgcacgccccagctcagggtggtcacgagggtgggccagggcacgggcagcttgccggtggtgcagatgaacttcagggtcagcttgccgtaggtggcatcgccctcgccctcgccggacacgctgaacttgtggccgtttacgtcgccgtccagctcgaccaggatgggcaccaccccggtgaacagctcctcgcccttgctcaccatggtggctctagagtaggcgccggtcacagcttggatctgtaacggcgcagaacagaaaacgaaacaaagacgtagagttgagcaagcagggtcaggcaaagcgtggagagccggctgagtctaggtaggctccaagggagcgccggacaaaggcccggtctcgacctgagctttaaacttacctagacggcggacgcagttcaggaggcaccacaggcgggaggcggcagaacgcgactcaaccggcgtggatggcggcctcaggtagggcggcgggcgcgtgaaggagagatgcgagcccctcgaagcttcagctgtgttctggcggcaaacccgttgcgaaaaagaacgttcacggcgactactgcacttatatacggttctcccccaccctcgggaaaaaggcggagccagtacacgacatcactttcccagtttaccccgcgccaccttctctaggcacccgttcaattgccgacccctccccccaacttctcggggactgtgggcgatgtgcgctctgcccactgacgggcaccggagccgtgtctgggtcctctccgggcatctctcctccctcacccaaccccatgccgtcttcactcgctgggttcccttttccttctccttctggggcctgtgccatctctcgtttcttaggatggccttctccgacggatgtctcccttgcgtcccgcctccccttcttgtaggcctgcatcatcaccgtttttctggacaaccccaaagtaccccgtctccctggctttagccacctctccatcctcttgctttctttgcctggacaccccgttctcctgtggattcgggtcacctctcactcctttcatttgggcagctcccctaccccccttacctctctagtctgtgctagctcttccagccccctgtcatggcatcttccaggggtccgagagctcagctagtcttcttcctccaacccgggcccctatgtccacttcaggacagcatgtttgctgcctccagggatcctgtgtccccgagctgggaccaccttatattcccagggccggttaatgtggctctggttctgggtacttttatctgtcccctccaccccacagtggggccactagggacaggattggtgacagaaaagccccatccttaggcctcctccttcctagtctcctgatattgggtctaacccccacctcctgttaggcagattccttatctggtgacacacccccatttcctggagccatctctctccttgccagaacctctaaggtttgcttacgatggagccagagaggatcctgggagggagagcttggcagggggtgggagggaaggggg

SEQ ID NO: 21 - DNA, 3012 bp, Artificial Sequence
ccctctcctgaacctgagccagctcccatagctcagtctggtctatctgcctggccctggccattgtcactttgcgctgccctcctctcgcccccgagtgcccttgctgtgccgccggaactctgccctctaacgctgccgtctctctcctgagtccggaccactttgagctctactggcttctgcgccgcctctggcccactgtttccccttcccaggcaggtcctgctttctctgacctgcattctctcccctgggcctgtgccgctttctgtctgcagcttgtggcctgggtcacctctacggctggcccagatccttccctgccgcctccttcaggttccgtcttcctccactccctcttccccttgctctctgctgtgttgctgcccaaggatgctctttccggagcacttccttctcggcgctgcaccacgtgatgtcctctgagcggatcctccccgtgtctgggtcctctccgggcatctctcctccctcacccaaccccatgccgtcttcactcgctgggttcccttttccttctccttctggggcctgtgccatctctcgtttcttaggatggccttctccgacggatgtctcccttgcgtcccgcctccccttcttgtaggcctgcatcatcaccgtttttctggacaaccccaaagtaccccgtctccctggctttagccacctctccatcctcttgctttctttgcctggacaccccgttctcctgtggattcgggtcacctctcactcctttcatttgggcagctcccctaccccccttacctctctaagatacattgatgagtttggacaaaccacaactagaatgcagtgaaaaaaatgctttatttgtgaaatttgtgatgctattgctttatttgtaaccattataagctgcaataaacaagttgtcgaggccgcggatccttcgaattctcacttgtacagctcgtccatgccgagagtgatcccggcggcggtcacgaactccagcaggaccatgtgatcgcgcttctcgttggggtctttgctcagcttggactgggtgctcaggtagtggttgtcgggcagcagcacggggccgtcgccgatgggggtgttctgctggtagtggtcggcgagctgcacgccgccgtcctcgatgttgtggcggatcttgaagttggccttgatgccgttcttctgcttgtcggcggtgatatagacgttgtcgctgaagtagttgtactccagcttgtgccccaggatgttgccgtcctccttgaagtcgatgcccttcagctcgatgcggttcaccagggtgtcgccctcgaacttcacctcggcgcgggtcttgtagttgccgtcgtccttgaagaagatggtgcgctcctggacgtagccttcgggcatggcggacttgaagaagtcgtgctgcttcatgtggtcggggtagcgggcgaagcactgcacgccccagctcagggtggtcacgagggtgggccagggcacgggcagcttgccggtggtgcagatgaacttcagggtcagcttgccgtaggtggcatcgccctcgccctcgccggacacgctgaacttgtggccgtttacgtcgccgtccagctcgaccaggatgggcaccaccccggtgaacagctcctcgcccttgctcaccatggtggctctagagtaggcgccggtcacagcttggatctgtaacggcgcagaacagaaaacgaaacaaagacgtagagttgagcaagcagggtcaggcaaagcgtggagagccggctgagtctaggtaggctccaagggagcgccggacaaaggcccggtctcgacctgagctttaaacttacctagacggcggacgcagttcaggaggcaccacaggcgggaggcggcagaacgcgactcaaccggcgtggatggcggcctcaggtagggcggcgggcgcgtgaaggagagatgcgagcccctcgaagcttcagctgtgttctggcggcaaacccgttgcgaaaaagaacgttcacggcgactactgcacttatatacggttctcccccaccctcgggaaaaaggcggagccagtacacgacatcactttcccagtttaccccgcgccaccttctctaggcacccgttcaattgccgacccctccccccaacttctcggggactgtgggcgatgtgcgctctgcccactgacgggcaccggagctagtctgtgctagctcttccagccccctgtcatggcatcttccaggggtccgagagctcagctagtcttcttcctccaacccgggcccctatgtccacttcaggacagcatgtttgctgcctccagggatcctgtgtccccgagctgggaccaccttatattcccagggccggttaatgtggctctggttctgggtacttttatctgtcccctccaccccacagtggggccactagggacaggattggtgacagaaaagccccatccttaggcctcctccttcctagtctcctgatattgggtctaacccccacctcctgttaggcagattccttatctggtgacacacccccatttcctggagccatctctctccttgccagaacctctaaggtttgcttacgatggagccagagaggatcctgggagggagagcttggcagggggtgggagggaagggggggatgcgtgacctgcccggttctcagtggccaccctgcgctaccctctcccagaacctgagctgctctgacgcggccgtctggtgcgtttcactgatcctggtgctgcagcttccttacacttcccaagaggagaagcagtttggaaaaacaaaatcagaataagttggtcctgagttctaactttggctcttcacctttctagtccccaatttatattgttcctccgtgcgtcagttttacctgtgagataaggccagtagccagccccgtcctggcagggctgtggtgaggaggggggtgtccgtgtggaaaactccctttgtgagaatggtgcgt

SEQ ID NO: 22 - DNA, 3012 bp, Artificial Sequence
gtgctgacccatgcagtcctccttaccatccctccctcgacttcccctcttccgatgttgagcccctccagccggtcctggactttgtctccttccctgccctgccctctcctgaacctgagccagctcccatagctcagtctggtctatctgcctggccctggccattgtcactttgcgctgccctcctctcgcccccgagtgcccttgctgtgccgccggaactctgccctctaacgctgccgtctctctcctgagtccggaccactttgagctctactggcttctgcgccgcctctggcccactgtttccccttcccaggcaggtcctgctttctctgacctgcattctctcccctgggcctgtgccgctttctgtctgcagcttgtggcctgggtcacctctacggctggcccagatccttccctgccgcctccttcaggttccgtcttcctccactccctcttccccttgctctctgctgtgttgctgcccaaggatgctctttccggagcacttccttctcggcgctgcaccacgtgatgtcctctgagcggatcctccccgtgtctgggtcctctccgggcatctctcctccctcacccaaccccatgccgtcttcactcgctgggttcccttttccttctccttctggggcctgtgccatctctcgtttcttaggatggccttctccgacggatgtctcccttgcgtcccgcctccccttcttgtaggcctgcatcatcaccgtttttctggacaaccccaaagtaccccgtctccctggctttagccaccttaagatacattgatgagtttggacaaaccacaactagaatgcagtgaaaaaaatgctttatttgtgaaatttgtgatgctattgctttatttgtaaccattataagctgcaataaacaagttgtcgaggccgcggatccttcgaattctcacttgtacagctcgtccatgccgagagtgatcccggcggcggtcacgaactccagcaggaccatgtgatcgcgcttctcgttggggtctttgctcagcttggactgggtgctcaggtagtggttgtcgggcagcagcacggggccgtcgccgatgggggtgttctgctggtagtggtcggcgagctgcacgccgccgtcctcgatgttgtggcggatcttgaagttggccttgatgccgttcttctgcttgtcggcggtgatatagacgttgtcgctgaagtagttgtactccagcttgtgccccaggatgttgccgtcctccttgaagtcgatgcccttcagctcgatgcggttcaccagggtgtcgccctcgaacttcacctcggcgcgggtcttgtagttgccgtcgtccttgaagaagatggtgcgctcctggacgtagccttcgggcatggcggacttgaagaagtcgtgctgcttcatgtggtcggggtagcgggcgaagcactgcacgccccagctcagggtggtcacgagggtgggccagggcacgggcagcttgccggtggtgcagatgaacttcagggtcagcttgccgtaggtggcatcgccctcgccctcgccggacacgctgaacttgtggccgtttacgtcgccgtccagctcgaccaggatgggcaccaccccggtgaacagctcctcgcccttgctcaccatggtggctctagagtaggcgccggtcacagcttggatctgtaacggcgcagaacagaaaacgaaacaaagacgtagagttgagcaagcagggtcaggcaaagcgtggagagccggctgagtctaggtaggctccaagggagcgccggacaaaggcccggtctcgacctgagctttaaacttacctagacggcggacgcagttcaggaggcaccacaggcgggaggcggcagaacgcgactcaaccggcgtggatggcggcctcaggtagggcggcgggcgcgtgaaggagagatgcgagcccctcgaagcttcagctgtgttctggcggcaaacccgttgcgaaaaagaacgttcacggcgactactgcacttatatacggttctcccccaccctcgggaaaaaggcggagccagtacacgacatcactttcccagtttaccccgcgccaccttctctaggcacccgttcaattgccgacccctccccccaacttctcggggactgtgggcgatgtgcgctctgcccactgacgggcaccggagcctccatcctcttgctttctttgcctggacaccccgttctcctgtggattcgggtcacctctcactcctttcatttgggcagctcccctaccccccttacctctctagtctgtgctagctcttccagccccctgtcatggcatcttccaggggtccgagagctcagctagtcttcttcctccaacccgggcccctatgtccacttcaggacagcatgtttgctgcctccagggatcctgtgtccccgagctgggaccaccttatattcccagggccggttaatgtggctctggttctgggtacttttatctgtcccctccaccccacagtggggccactagggacaggattggtgacagaaaagccccatccttaggcctcctccttcctagtctcctgatattgggtctaacccccacctcctgttaggcagattccttatctggtgacacacccccatttcctggagccatctctctccttgccagaacctctaaggtttgcttacgatggagccagagaggatcctgggagggagagcttggcagggggtgggagggaagggggggatgcgtgacctgcccggttctcagtggccaccctgcgctaccctctcccagaacctgagctgctctgacgcggccgtctggtgcgtttcactgatcctggtgctgcagcttccttacacttcccaagaggagaagcagtttggaaaaacaaaatcagaataagttggtcctgagttctaactttggctcttcacctttctagtccccaatttatattgttcctccgtgcgtc

SEQ ID NO: 23 - DNA, 3012 bp, Artificial Sequence
ttttgcaggtgaaattcctgagatgtaaggagctgctgtgacttgctcaaggccttatatcgagtaaacggtagtgctggggcttagacgcaggtgttctgatttatagttcaaaacctctatcaatgagagagcaatctcctggtaatgtgatagatttcccaacttaatgccaacataccataaacctcccattctgctaatgcccagcctaagttggggagaccactccagattccaagatgtacagtttgctttgctgggcctttttcccatgcctgcctttactctgccagagttatattgctggggttttgaagaagatcctattaaataaaagaataagcagtattattaagtagccctgcatttcaggtttccttgagtggcaggccaggcctggccgtgaacgttcactgaaatcatggcctcttggccaagattgatagcttgtgcctgtccctgagtcccagtccatcacgagcagctggtttctaagatgctatttcccgtataaagcatgagaccgtgacttgccagccccacagagccccgcccttgtccatcactggcatctggactccagcctgggttggggcaaagagggaaatgagatcatgtcctaaccctgatcctcttgtcccacagatatccagaaccctgaccctgccgtgtaccagctgagagactctaaatccagtgacaagtctgtctgcctattcaccgattttgattctcaaacaaatgtgtcacaaagtaaggattctgatgtgtatatcacagacaaaactgtgctagactaagatacattgatgagtttggacaaaccacaactagaatgcagtgaaaaaaatgctttatttgtgaaatttgtgatgctattgctttatttgtaaccattataagctgcaataaacaagttgtcgaggccgcggatccttcgaattctcacttgtacagctcgtccatgccgagagtgatcccggcggcggtcacgaactccagcaggaccatgtgatcgcgcttctcgttggggtctttgctcagcttggactgggtgctcaggtagtggttgtcgggcagcagcacggggccgtcgccgatgggggtgttctgctggtagtggtcggcgagctgcacgccgccgtcctcgatgttgtggcggatcttgaagttggccttgatgccgttcttctgcttgtcggcggtgatatagacgttgtcgctgaagtagttgtactccagcttgtgccccaggatgttgccgtcctccttgaagtcgatgcccttcagctcgatgcggttcaccagggtgtcgccctcgaacttcacctcggcgcgggtcttgtagttgccgtcgtccttgaagaagatggtgcgctcctggacgtagccttcgggcatggcggacttgaagaagtcgtgctgcttcatgtggtcggggtagcgggcgaagcactgcacgccccagctcagggtggtcacgagggtgggccagggcacgggcagcttgccggtggtgcagatgaacttcagggtcagcttgccgtaggtggcatcgccctcgccctcgccggacacgctgaacttgtggccgtttacgtcgccgtccagctcgaccaggatgggcaccaccccggtgaacagctcctcgcccttgctcaccatggtggctctagagtaggcgccggtcacagcttggatctgtaacggcgcagaacagaaaacgaaacaaagacgtagagttgagcaagcagggtcaggcaaagcgtggagagccggctgagtctaggtaggctccaagggagcgccggacaaaggcccggtctcgacctgagctttaaacttacctagacggcggacgcagttcaggaggcaccacaggcgggaggcggcagaacgcgactcaaccggcgtggatggcggcctcaggtagggcggcgggcgcgtgaaggagagatgcgagcccctcgaagcttcagctgtgttctggcggcaaacccgttgcgaaaaagaacgttcacggcgactactgcacttatatacggttctcccccaccctcgggaaaaaggcggagccagtacacgacatcactttcccagtttaccccgcgccaccttctctaggcacccgttcaattgccgacccctccccccaacttctcggggactgtgggcgatgtgcgctctgcccactgacgggcaccggagcatgaggtctatggacttcaagagcaacagtgctgtggcctggagcaacaaatctgactttgcatgtgcaaacgccttcaacaacagcattattccagaagacaccttcttccccagcccaggtaagggcagctttggtgccttcgcaggctgtttccttgcttcaggaatggccaggttctgcccagagctctggtcaatgatgtctaaaactcctctgattggtggtctcggccttatccattgccaccaaaaccctctttttactaagaaacagtgagccttgttctggcagtccagagaatgacacgggaaaaaagcagatgaagagaaggtggcaggagagggcacgtggcccagcctcagtctctccaactgagttcctgcctgcctgcctttgctcagactgtttgccccttactgctcttctaggcctcattctaagccccttctccaagttgcctctccttatttctccctgtctgccaaaaaatctttcccagctcactaagtcagtctcacgcagtcactcattaacccaccaatcactgattgtgccggcacatgaatgcaccaggtgttgaagtggaggaattaaaaagtcagatgaggggtgtgcccagaggaagcaccattctagttgggggagcccatctgtcagctgggaaaagtccaaataacttcagattggaatgtgttttaactcagggttgagaaaacagctaccttcaggacaaaagtcagggaagggctctctgaagaaatgctacttgaagataccagccctaccaagggcaggga

SEQ ID NO: 24 - DNA, 3012 bp, Artificial Sequence
tgtgacttgctcaaggccttatatcgagtaaacggtagtgctggggcttagacgcaggtgttctgatttatagttcaaaacctctatcaatgagagagcaatctcctggtaatgtgatagatttcccaacttaatgccaacataccataaacctcccattctgctaatgcccagcctaagttggggagaccactccagattccaagatgtacagtttgctttgctgggcctttttcccatgcctgcctttactctgccagagttatattgctggggttttgaagaagatcctattaaataaaagaataagcagtattattaagtagccctgcatttcaggtttccttgagtggcaggccaggcctggccgtgaacgttcactgaaatcatggcctcttggccaagattgatagcttgtgcctgtccctgagtcccagtccatcacgagcagctggtttctaagatgctatttcccgtataaagcatgagaccgtgacttgccagccccacagagccccgcccttgtccatcactggcatctggactccagcctgggttggggcaaagagggaaatgagatcatgtcctaaccctgatcctcttgtcccacagatatccagaaccctgaccctgccgtgtaccagctgagagactctaaatccagtgacaagtctgtctgcctattcaccgattttgattctcaaacaaatgtgtcacaaagtaaggattctgatgtgtatatcacagacaaaactgtgctagacatgaggtctatggacttcaagagcaacagtgctgtgtaagatacattgatgagtttggacaaaccacaactagaatgcagtgaaaaaaatgctttatttgtgaaatttgtgatgctattgctttatttgtaaccattataagctgcaataaacaagttgtcgaggccgcggatccttcgaattctcacttgtacagctcgtccatgccgagagtgatcccggcggcggtcacgaactccagcaggaccatgtgatcgcgcttctcgttggggtctttgctcagcttggactgggtgctcaggtagtggttgtcgggcagcagcacggggccgtcgccgatgggggtgttctgctggtagtggtcggcgagctgcacgccgccgtcctcgatgttgtggcggatcttgaagttggccttgatgccgttcttctgcttgtcggcggtgatatagacgttgtcgctgaagtagttgtactccagcttgtgccccaggatgttgccgtcctccttgaagtcgatgcccttcagctcgatgcggttcaccagggtgtcgccctcgaacttcacctcggcgcgggtcttgtagttgccgtcgtccttgaagaagatggtgcgctcctggacgtagccttcgggcatggcggacttgaagaagtcgtgctgcttcatgtggtcggggtagcgggcgaagcactgcacgccccagctcagggtggtcacgagggtgggccagggcacgggcagcttgccggtggtgcagatgaacttcagggtcagcttgccgtaggtggcatcgccctcgccctcgccggacacgctgaacttgtggccgtttacgtcgccgtccagctcgaccaggatgggcaccaccccggtgaacagctcctcgcccttgctcaccatggtggctctagagtaggcgccggtcacagcttggatctgtaacggcgcagaacagaaaacgaaacaaagacgtagagttgagcaagcagggtcaggcaaagcgtggagagccggctgagtctaggtaggctccaagggagcgccggacaaaggcccggtctcgacctgagctttaaacttacctagacggcggacgcagttcaggaggcaccacaggcgggaggcggcagaacgcgactcaaccggcgtggatggcggcctcaggtagggcggcgggcgcgtgaaggagagatgcgagcccctcgaagcttcagctgtgttctggcggcaaacccgttgcgaaaaagaacgttcacggcgactactgcacttatatacggttctcccccaccctcgggaaaaaggcggagccagtacacgacatcactttcccagtttaccccgcgccaccttctctaggcacccgttcaattgccgacccctccccccaacttctcggggactgtgggcgatgtgcgctctgcccactgacgggcaccggagcgcctggagcaacaaatctgactttgcatgtgcaaacgccttcaacaacagcattattccagaagacaccttcttccccagcccaggtaagggcagctttggtgccttcgcaggctgtttccttgcttcaggaatggccaggttctgcccagagctctggtcaatgatgtctaaaactcctctgattggtggtctcggccttatccattgccaccaaaaccctctttttactaagaaacagtgagccttgttctggcagtccagagaatgacacgggaaaaaagcagatgaagagaaggtggcaggagagggcacgtggcccagcctcagtctctccaactgagttcctgcctgcctgcctttgctcagactgtttgccccttactgctcttctaggcctcattctaagccccttctccaagttgcctctccttatttctccctgtctgccaaaaaatctttcccagctcactaagtcagtctcacgcagtcactcattaacccaccaatcactgattgtgccggcacatgaatgcaccaggtgttgaagtggaggaattaaaaagtcagatgaggggtgtgcccagaggaagcaccattctagttgggggagcccatctgtcagctgggaaaagtccaaataacttcagattggaatgtgttttaactcagggttgagaaaacagctaccttcaggacaaaagtcagggaagggctctctgaagaaatgctacttgaagataccagccctaccaagggcagggagaggaccctatagaggcctgggacaggagctcaatg

SEQ ID NO: 25 - DNA, 3012 bp, Artificial Sequence
gtcagtggctccaactaacatttgtttggtactttacagtttattaaatagatgtttatatggagaagctctcatttctttctcagaagagcctggctaggaaggtggatgaggcaccatattcattttgcaggtgaaattcctgagatgtaaggagctgctgtgacttgctcaaggccttatatcgagtaaacggtagtgctggggcttagacgcaggtgttctgatttatagttcaaaacctctatcaatgagagagcaatctcctggtaatgtgatagatttcccaacttaatgccaacataccataaacctcccattctgctaatgcccagcctaagttggggagaccactccagattccaagatgtacagtttgctttgctgggcctttttcccatgcctgcctttactctgccagagttatattgctggggttttgaagaagatcctattaaataaaagaataagcagtattattaagtagccctgcatttcaggtttccttgagtggcaggccaggcctggccgtgaacgttcactgaaatcatggcctcttggccaagattgatagcttgtgcctgtccctgagtcccagtccatcacgagcagctggtttctaagatgctatttcccgtataaagcatgagaccgtgacttgccagccccacagagccccgcccttgtccatcactggcatctggactccagcctgggttggggcaaagagggaaatgagatcatgtcctaaccctgatcctcttgtcccacagatatccagaaccctgaccctgccgtgttaagatacattgatgagtttggacaaaccacaactagaatgcagtgaaaaaaatgctttatttgtgaaatttgtgatgctattgctttatttgtaaccattataagctgcaataaacaagttgtcgaggccgcggatccttcgaattctcacttgtacagctcgtccatgccgagagtgatcccggcggcggtcacgaactccagcaggaccatgtgatcgcgcttctcgttggggtctttgctcagcttggactgggtgctcaggtagtggttgtcgggcagcagcacggggccgtcgccgatgggggtgttctgctggtagtggtcggcgagctgcacgccgccgtcctcgatgttgtggcggatcttgaagttggccttgatgccgttcttctgcttgtcggcggtgatatagacgttgtcgctgaagtagttgtactccagcttgtgccccaggatgttgccgtcctccttgaagtcgatgcccttcagctcgatgcggttcaccagggtgtcgccctcgaacttcacctcggcgcgggtcttgtagttgccgtcgtccttgaagaagatggtgcgctcctggacgtagccttcgggcatggcggacttgaagaagtcgtgctgcttcatgtggtcggggtagcgggcgaagcactgcacgccccagctcagggtggtcacgagggtgggccagggcacgggcagcttgccggtggtgcagatgaacttcagggtcagcttgccgtaggtggcatcgccctcgccctcgccggacacgctgaacttgtggccgtttacgtcgccgtccagctcgaccaggatgggcaccaccccggtgaacagctcctcgcccttgctcaccatggtggctctagagtaggcgccggtcacagcttggatctgtaacggcgcagaacagaaaacgaaacaaagacgtagagttgagcaagcagggtcaggcaaagcgtggagagccggctgagtctaggtaggctccaagggagcgccggacaaaggcccggtctcgacctgagctttaaacttacctagacggcggacgcagttcaggaggcaccacaggcgggaggcggcagaacgcgactcaaccggcgtggatggcggcctcaggtagggcggcgggcgcgtgaaggagagatgcgagcccctcgaagcttcagctgtgttctggcggcaaacccgttgcgaaaaagaacgttcacggcgactactgcacttatatacggttctcccccaccctcgggaaaaaggcggagccagtacacgacatcactttcccagtttaccccgcgccaccttctctaggcacccgttcaattgccgacccctccccccaacttctcggggactgtgggcgatgtgcgctctgcccactgacgggcaccggagcaccagctgagagactctaaatccagtgacaagtctgtctgcctattcaccgattttgattctcaaacaaatgtgtcacaaagtaaggattctgatgtgtatatcacagacaaaactgtgctagacatgaggtctatggacttcaagagcaacagtgctgtggcctggagcaacaaatctgactttgcatgtgcaaacgccttcaacaacagcattattccagaagacaccttcttccccagcccaggtaagggcagctttggtgccttcgcaggctgtttccttgcttcaggaatggccaggttctgcccagagctctggtcaatgatgtctaaaactcctctgattggtggtctcggccttatccattgccaccaaaaccctctttttactaagaaacagtgagccttgttctggcagtccagagaatgacacgggaaaaaagcagatgaagagaaggtggcaggagagggcacgtggcccagcctcagtctctccaactgagttcctgcctgcctgcctttgctcagactgtttgccccttactgctcttctaggcctcattctaagccccttctccaagttgcctctccttatttctccctgtctgccaaaaaatctttcccagctcactaagtcagtctcacgcagtcactcattaacccaccaatcactgattgtgccggcacatgaatgcaccaggtgttgaagtggaggaattaaaaagtcagatgaggggtgtgcccagaggaagcaccattctagttgggggagcccatctgtcagctgggaaaagtccaa

SEQ ID NO: 26 - DNA, 3012 bp, Artificial Sequence
cgctggaagctctaaagccctagcagttactgcttttactattagtggtcgtttttttctcccccccgccccccgacaaatcaacagaacaaagaaaattacctaaacagcaaggacatagggaggaacttcttggcacagaactttccaaacactttttcctgaagggatacaagaagcaagaaaggtactctttcactaggaccttctctgagctgtcctcaggatgcttttgggactatttttcttacccagagaatggagaaaccctgcagggaattcccaagctgtagttataaacagaagttctccttctgctaggtagcattcaaagatcttaatcttctgggtttccgttttctcgaatgaaaaatgcaggtccgagcagttaactggctggggcaccattagcaagtcacttagcatctctggggccagtctgcaaagcgagggggcagccttaatgtgcctccagcctgaagtcctagaatgagcgcccggtgtcccaagctggggcgcgcaccccagatcggagggcgccgatgtacagacagcaaactcacccagtctagtgcatgccttcttaaacatcacgagactctaagaaaaggaaactgaaaacgggaaagtccctctctctaacctggcactgcgtcgctggcttggagacaggtgacggtccctgcgggccttgtcctgattggctgggcacgcgtttaatataagtggaggcgtcgcgctggcgggcattcctgaagctgacagcattcgggccgagatgtctcgctccgtggccttagtaagatacattgatgagtttggacaaaccacaactagaatgcagtgaaaaaaatgctttatttgtgaaatttgtgatgctattgctttatttgtaaccattataagctgcaataaacaagttgtcgaggccgcggatccttcgaattctcacttgtacagctcgtccatgccgagagtgatcccggcggcggtcacgaactccagcaggaccatgtgatcgcgcttctcgttggggtctttgctcagcttggactgggtgctcaggtagtggttgtcgggcagcagcacggggccgtcgccgatgggggtgttctgctggtagtggtcggcgagctgcacgccgccgtcctcgatgttgtggcggatcttgaagttggccttgatgccgttcttctgcttgtcggcggtgatatagacgttgtcgctgaagtagttgtactccagcttgtgccccaggatgttgccgtcctccttgaagtcgatgcccttcagctcgatgcggttcaccagggtgtcgccctcgaacttcacctcggcgcgggtcttgtagttgccgtcgtccttgaagaagatggtgcgctcctggacgtagccttcgggcatggcggacttgaagaagtcgtgctgcttcatgtggtcggggtagcgggcgaagcactgcacgccccagctcagggtggtcacgagggtgggccagggcacgggcagcttgccggtggtgcagatgaacttcagggtcagcttgccgtaggtggcatcgccctcgccctcgccggacacgctgaacttgtggccgtttacgtcgccgtccagctcgaccaggatgggcaccaccccggtgaacagctcctcgcccttgctcaccatggtggctctagagtaggcgccggtcacagcttggatctgtaacggcgcagaacagaaaacgaaacaaagacgtagagttgagcaagcagggtcaggcaaagcgtggagagccggctgagtctaggtaggctccaagggagcgccggacaaaggcccggtctcgacctgagctttaaacttacctagacggcggacgcagttcaggaggcaccacaggcgggaggcggcagaacgcgactcaaccggcgtggatggcggcctcaggtagggcggcgggcgcgtgaaggagagatgcgagcccctcgaagcttcagctgtgttctggcggcaaacccgttgcgaaaaagaacgttcacggcgactactgcacttatatacggttctcccccaccctcgggaaaaaggcggagccagtacacgacatcactttcccagtttaccccgcgccaccttctctaggcacccgttcaattgccgacccctccccccaacttctcggggactgtgggcgatgtgcgctctgcccactgacgggcaccggagcctgtgctcgcgctactctctctttctggcctggaggctatccagcgtgagtctctcctaccctcccgctctggtccttcctctcccgctctgcaccctctgtggccctcgctgtgctctctcgctccgtgacttcccttctccaagttctccttggtggcccgccgtggggctagtccagggctggatctcggggaagcggcggggtggcctgggagtggggaagggggtgcgcacccgggacgcgcgctacttgcccctttcggcggggagcaggggagacctttggcctacggcgacgggagggtcgggacaaagtttagggcgtcgataagcgtcagagcgccgaggttgggggagggtttctcttccgctctttcgcggggcctctggctcccccagcgcagctggagtgggggacgggtaggctcgtcccaaaggcgcggcgctgaggtttgtgaacgcgtggaggggcgcttggggtctgggggaggcgtcgcccgggtaagcctgtctgctgcggctctgcttcccttagactggagagctgtggacttcgtctaggcgcccgctaagttcgcatgtcctagcacctctgggtctatgtggggccacaccgtggggaggaaacagcacgcgacgtttgtagaatgcttggctgtgatacaaagcggtttcgaataattaacttatttgttcccatcacatgtcacttttaaaaaattataagaactacccgttattgacatctttctgtgtgccaaggactttatgtgctttgcgtcatttaattttgaaaac

SEQ ID NO: 27 - DNA, 2562 bp, Artificial Sequence
gacggatgtctcccttgcgtcccgcctccccttcttgtaggcctgcatcatcaccgtttttctggacaaccccaaagtaccccgtctccctggctttagccacctctccatcctcttgctttctttgcctggacaccccgttctcctgtggattcgggtcacctctcactcctttcatttgggcagctcccctaccccccttacctctctaagatacattgatgagtttggacaaaccacaactagaatgcagtgaaaaaaatgctttatttgtgaaatttgtgatgctattgctttatttgtaaccattataagctgcaataaacaagttgtcgaggccgcggatccttcgaattcttagcgagggggcagggcctgcatgtgaagggcgtcgtaggtgtccttggtggctgtactgagaccctggtaaaggccatcgtgccccttgcccctccggcgctcgcctttcatcccaatctcactgtaggcctccgccatcttatctttctgcagttcattgtacaggccttcctgagggttcttccttctcggctttccccccatctcagggtcccggccacgtctcttgtccaaaacatcgtactcctctcttcgtcctagattgagctcgttatagagctggttctggccctgcttgtacgcgggggcgtctgcgctcctgctgaacttcactctcagttcacatcctccttcttcttcttctggaaatcggcagctacagccatcttcctcttgagtagtttgtactggtctcataaatggttgtttgaatatatacaggagtttctttctgccccgtttgcagtaaagggtgataaccagtgacaggagaaggaccccacaagtcccggccaagggcgcccagatgtagatatcacaggcgaagtccagccccctcgtgtgcactgcgccccccgccgctggccggcacgcctctgggcgcagggacaggggctgcgacgcgatggtgggcgccggtgttggtggtcgcggcgctggcgtcgtggttgaggagacggtgactgaggttccttggccccagtagtccatagcatagctaccaccgtagtaataatgtttggcacagtagtaaatggctgtgtcatcagtttgcagactgttcatttttaagaaaacttggctcttggagttgtccttgatgatggtcagtctggatttgagagctgaattatagtatgtggtttcactaccccatattactcccagccactccagaccctttcgtggaggctggcgaatccagcttacaccatagtcgggtaatgagacccctgagacagtgcatgtgacggacaggctctgtgagggcgccaccaggccaggtcctgactcctgcagtttcacctcagatccgccgccacccgacccaccaccgcccgagccaccgccacctgtgatctccagcttggtcccccctccgaacgtgtacggaagcgtattaccctgttggcaaaagtaagtggcaatatcttcttgctccaggttgctaatggtgagagaataatctgttccagacccactgccactgaaccttgatgggactcctgagtgtaatcttgatgtatggtagatcaggagtttaacagttccatctggtttctgctgataccaatttaaatatttactaatgtcctgacttgccctgcaactgatggtgactctgtctcccagagaggcagacagggaggatgtagtctgtgtcatctggatgtccggcctggcggcgtggagcagcaaggccagcggcaggagcaaggcggtcactggtaaggccatggtggctctagagtaggcgccggtcacagcttggatctgtaacggcgcagaacagaaaacgaaacaaagacgtagagttgagcaagcagggtcaggcaaagcgtggagagccggctgagtctaggtaggctccaagggagcgccggacaaaggcccggtctcgacctgagctttaaacttacctagacggcggacgcagttcaggaggcaccacaggcgggaggcggcagaacgcgactcaaccggcgtggatggcggcctcaggtagggcggcgggcgcgtgaaggagagatgcgagcccctcgaagcttcagctgtgttctggcggcaaacccgttgcgaaaaagaacgttcacggcgactactgcacttatatacggttctcccccaccctcgggaaaaaggcggagccagtacacgacatcactttcccagtttaccccgcgccaccttctctaggcacccgttcaattgccgacccctccccccaacttctcggggactgtgggcgatgtgcgctctgcccactgacgggcaccggagctagtctgtgctagctcttccagccccctgtcatggcatcttccaggggtccgagagctcagctagtcttcttcctccaacccgggcccctatgtccacttcaggacagcatgtttgctgcctccagggatcctgtgtccccgagctgggaccaccttatattcccagggccggttaatgtggctctggttctgggtactt

SEQ ID NO: 28 - DNA, 2953 bp, Artificial Sequence
tctttccggagcacttccttctcggcgctgcaccacgtgatgtcctctgagcggatcctccccgtgtctgggtcctctccgggcatctctcctccctcacccaaccccatgccgtcttcactcgctgggttcccttttccttctccttctggggcctgtgccatctctcgtttcttaggatggccttctccgacggatgtctcccttgcgtcccgcctccccttcttgtaggcctgcatcatcaccgtttttctggacaaccccaaagtaccccgtctccctggctttagccacctctccatcctcttgctttctttgcctggacaccccgttctcctgtggattcgggtcacctctcactcctttcatttgggcagctcccctaccccccttacctctctaagatacattgatgagtttggacaaaccacaactagaatgcagtgaaaaaaatgctttatttgtgaaatttgtgatgctattgctttatttgtaaccattataagctgcaataaacaagttgtcgaggccgcggatccttcgaattcttagcgagggggcagggcctgcatgtgaagggcgtcgtaggtgtccttggtggctgtactgagaccctggtaaaggccatcgtgccccttgcccctccggcgctcgcctttcatcccaatctcactgtaggcctccgccatcttatctttctgcagttcattgtacaggccttcctgagggttcttccttctcggctttccccccatctcagggtcccggccacgtctcttgtccaaaacatcgtactcctctcttcgtcctagattgagctcgttatagagctggttctggccctgcttgtacgcgggggcgtctgcgctcctgctgaacttcactctcagttcacatcctccttcttcttcttctggaaatcggcagctacagccatcttcctcttgagtagtttgtactggtctcataaatggttgtttgaatatatacaggagtttctttctgccccgtttgcagtaaagggtgataaccagtgacaggagaaggaccccacaagtcccggccaagggcgcccagatgtagatatcacaggcgaagtccagccccctcgtgtgcactgcgccccccgccgctggccggcacgcctctgggcgcagggacaggggctgcgacgcgatggtgggcgccggtgttggtggtcgcggcgctggcgtcgtggttgaggagacggtgactgaggttccttggccccagtagtccatagcatagctaccaccgtagtaataatgtttggcacagtagtaaatggctgtgtcatcagtttgcagactgttcatttttaagaaaacttggctcttggagttgtccttgatgatggtcagtctggatttgagagctgaattatagtatgtggtttcactaccccatattactcccagccactccagaccctttcgtggaggctggcgaatccagcttacaccatagtcgggtaatgagacccctgagacagtgcatgtgacggacaggctctgtgagggcgccaccaggccaggtcctgactcctgcagtttcacctcagatccgccgccacccgacccaccaccgcccgagccaccgccacctgtgatctccagcttggtcccccctccgaacgtgtacggaagcgtattaccctgttggcaaaagtaagtggcaatatcttcttgctccaggttgctaatggtgagagaataatctgttccagacccactgccactgaaccttgatgggactcctgagtgtaatcttgatgtatggtagatcaggagtttaacagttccatctggtttctgctgataccaatttaaatatttactaatgtcctgacttgccctgcaactgatggtgactctgtctcccagagaggcagacagggaggatgtagtctgtgtcatctggatgtccggcctggcggcgtggagcagcaaggccagcggcaggagcaaggcggtcactggtaaggccatggtggctctagagtaggcgccggtcacagcttggatctgtaacggcgcagaacagaaaacgaaacaaagacgtagagttgagcaagcagggtcaggcaaagcgtggagagccggctgagtctaggtaggctccaagggagcgccggacaaaggcccggtctcgacctgagctttaaacttacctagacggcggacgcagttcaggaggcaccacaggcgggaggcggcagaacgcgactcaaccggcgtggatggcggcctcaggtagggcggcgggcgcgtgaaggagagatgcgagcccctcgaagcttcagctgtgttctggcggcaaacccgttgcgaaaaagaacgttcacggcgactactgcacttatatacggttctcccccaccctcgggaaaaaggcggagccagtacacgacatcactttcccagtttaccccgcgccaccttctctaggcacccgttcaattgccgacccctccccccaacttctcggggactgtgggcgatgtgcgctctgcccactgacgggcaccggagctagtctgtgctagctcttccagccccctgtcatggcatcttccaggggtccgagagctcagctagtcttcttcctccaacccgggcccctatgtccacttcaggacagcatgtttgctgcctccagggatcctgtgtccccgagctgggaccaccttatattcccagggccggttaatgtggctctggttctgggtacttttatctgtcccctccaccccacagtggggccactagggacaggattggtgacagaaaagccccatccttaggcctcctccttcctagtctcctgatattgggtctaacccccacctcctgttaggcagattccttatctggtgacacacccccatttcctggagccatctctctccttgccagaacctctaaggtttgct

SEQ ID NO: 29 - DNA, 3753 bp, Artificial Sequence
ccctctcctgaacctgagccagctcccatagctcagtctggtctatctgcctggccctggccattgtcactttgcgctgccctcctctcgcccccgagtgcccttgctgtgccgccggaactctgccctctaacgctgccgtctctctcctgagtccggaccactttgagctctactggcttctgcgccgcctctggcccactgtttccccttcccaggcaggtcctgctttctctgacctgcattctctcccctgggcctgtgccgctttctgtctgcagcttgtggcctgggtcacctctacggctggcccagatccttccctgccgcctccttcaggttccgtcttcctccactccctcttccccttgctctctgctgtgttgctgcccaaggatgctctttccggagcacttccttctcggcgctgcaccacgtgatgtcctctgagcggatcctccccgtgtctgggtcctctccgggcatctctcctccctcacccaaccccatgccgtcttcactcgctgggttcccttttccttctccttctggggcctgtgccatctctcgtttcttaggatggccttctccgacggatgtctcccttgcgtcccgcctccccttcttgtaggcctgcatcatcaccgtttttctggacaaccccaaagtaccccgtctccctggctttagccacctctccatcctcttgctttctttgcctggacaccccgttctcctgtggattcgggtcacctctcactcctttcatttgggcagctcccctaccccccttacctctctaagatacattgatgagtttggacaaaccacaactagaatgcagtgaaaaaaatgctttatttgtgaaatttgtgatgctattgctttatttgtaaccattataagctgcaataaacaagttgtcgaggccgcggatccttcgaattcttagcgagggggcagggcctgcatgtgaagggcgtcgtaggtgtccttggtggctgtactgagaccctggtaaaggccatcgtgccccttgcccctccggcgctcgcctttcatcccaatctcactgtaggcctccgccatcttatctttctgcagttcattgtacaggccttcctgagggttcttccttctcggctttccccccatctcagggtcccggccacgtctcttgtccaaaacatcgtactcctctcttcgtcctagattgagctcgttatagagctggttctggccctgcttgtacgcgggggcgtctgcgctcctgctgaacttcactctcagttcacatcctccttcttcttcttctggaaatcggcagctacagccatcttcctcttgagtagtttgtactggtctcataaatggttgtttgaatatatacaggagtttctttctgccccgtttgcagtaaagggtgataaccagtgacaggagaaggaccccacaagtcccggccaagggcgcccagatgtagatatcacaggcgaagtccagccccctcgtgtgcactgcgccccccgccgctggccggcacgcctctgggcgcagggacaggggctgcgacgcgatggtgggcgccggtgttggtggtcgcggcgctggcgtcgtggttgaggagacggtgactgaggttccttggccccagtagtccatagcatagctaccaccgtagtaataatgtttggcacagtagtaaatggctgtgtcatcagtttgcagactgttcatttttaagaaaacttggctcttggagttgtccttgatgatggtcagtctggatttgagagctgaattatagtatgtggtttcactaccccatattactcccagccactccagaccctttcgtggaggctggcgaatccagcttacaccatagtcgggtaatgagacccctgagacagtgcatgtgacggacaggctctgtgagggcgccaccaggccaggtcctgactcctgcagtttcacctcagatccgccgccacccgacccaccaccgcccgagccaccgccacctgtgatctccagcttggtcccccctccgaacgtgtacggaagcgtattaccctgttggcaaaagtaagtggcaatatcttcttgctccaggttgctaatggtgagagaataatctgttccagacccactgccactgaaccttgatgggactcctgagtgtaatcttgatgtatggtagatcaggagtttaacagttccatctggtttctgctgataccaatttaaatatttactaatgtcctgacttgccctgcaactgatggtgactctgtctcccagagaggcagacagggaggatgtagtctgtgtcatctggatgtccggcctggcggcgtggagcagcaaggccagcggcaggagcaaggcggtcactggtaaggccatggtggctctagagtaggcgccggtcacagcttggatctgtaacggcgcagaacagaaaacgaaacaaagacgtagagttgagcaagcagggtcaggcaaagcgtggagagccggctgagtctaggtaggctccaagggagcgccggacaaaggcccggtctcgacctgagctttaaacttacctagacggcggacgcagttcaggaggcaccacaggcgggaggcggcagaacgcgactcaaccggcgtggatggcggcctcaggtagggcggcgggcgcgtgaaggagagatgcgagcccctcgaagcttcagctgtgttctggcggcaaacccgttgcgaaaaagaacgttcacggcgactactgcacttatatacggttctcccccaccctcgggaaaaaggcggagccagtacacgacatcactttcccagtttaccccgcgccaccttctctaggcacccgttcaattgccgacccctccccccaacttctcggggactgtgggcgatgtgcgctctgcccactgacgggcaccggagctagtctgtgctagctcttccagccccctgtcatggcatcttccaggggtccgagagctcagctagtcttcttcctccaacccgggcccctatgtccacttcaggacagcatgtttgctgcctccagggatcctgtgtccccgagctgggaccaccttatattcccagggccggttaatgtggctctggttctgggtacttttatctgtcccctccaccccacagtggggccactagggacaggattggtgacagaaaagccccatccttaggcctcctccttcctagtctcctgatattgggtctaacccccacctcctgttaggcagattccttatctggtgacacacccccatttcctggagccatctctctccttgccagaacctctaaggtttgcttacgatggagccagagaggatcctgggagggagagcttggcagggggtgggagggaagggggggatgcgtgacctgcccggttctcagtggccaccctgcgctaccctctcccagaacctgagctgctctgacgcggccgtctggtgcgtttcactgatcctggtgctgcagcttccttacacttcccaagaggagaagcagtttggaaaaacaaaatcagaataagttggtcctgagttctaactttggctcttcacctttctagtccccaatttatattgttcctccgtgcgtcagttttacctgtgagataaggccagtagccagccccgtcctggcagggctgtggtgaggaggggggtgtccgtgtggaaaactccctttgtgagaatggtgcgt

SEQ ID NO: 30 - DNA, 2553 bp, Artificial Sequence
accccctcctcacccctcctcccccagcactgcctctgtcactctcgcccacgtggatgtggaggaagagggggcgggagcaaggggcgggcaccctcccttcaacctgacctgggacagtttcccttccgctcacctccgcctgagcagtggagaaggcggcactctggtggggctgctccaggcatgcagatcccacataagatacattgatgagtttggacaaaccacaactagaatgcagtgaaaaaaatgctttatttgtgaaatttgtgatgctattgctttatttgtaaccattataagctgcaataaacaagttgtcgaggccgcggatccttcgaattcttagcgagggggcagggcctgcatgtgaagggcgtcgtaggtgtccttggtggctgtactgagaccctggtaaaggccatcgtgccccttgcccctccggcgctcgcctttcatcccaatctcactgtaggcctccgccatcttatctttctgcagttcattgtacaggccttcctgagggttcttccttctcggctttccccccatctcagggtcccggccacgtctcttgtccaaaacatcgtactcctctcttcgtcctagattgagctcgttatagagctggttctggccctgcttgtacgcgggggcgtctgcgctcctgctgaacttcactctcagttcacatcctccttcttcttcttctggaaatcggcagctacagccatcttcctcttgagtagtttgtactggtctcataaatggttgtttgaatatatacaggagtttctttctgccccgtttgcagtaaagggtgataaccagtgacaggagaaggaccccacaagtcccggccaagggcgcccagatgtagatatcacaggcgaagtccagccccctcgtgtgcactgcgccccccgccgctggccggcacgcctctgggcgcagggacaggggctgcgacgcgatggtgggcgccggtgttggtggtcgcggcgctggcgtcgtggttgaggagacggtgactgaggttccttggccccagtagtccatagcatagctaccaccgtagtaataatgtttggcacagtagtaaatggctgtgtcatcagtttgcagactgttcatttttaagaaaacttggctcttggagttgtccttgatgatggtcagtctggatttgagagctgaattatagtatgtggtttcactaccccatattactcccagccactccagaccctttcgtggaggctggcgaatccagcttacaccatagtcgggtaatgagacccctgagacagtgcatgtgacggacaggctctgtgagggcgccaccaggccaggtcctgactcctgcagtttcacctcagatccgccgccacccgacccaccaccgcccgagccaccgccacctgtgatctccagcttggtcccccctccgaacgtgtacggaagcgtattaccctgttggcaaaagtaagtggcaatatcttcttgctccaggttgctaatggtgagagaataatctgttccagacccactgccactgaaccttgatgggactcctgagtgtaatcttgatgtatggtagatcaggagtttaacagttccatctggtttctgctgataccaatttaaatatttactaatgtcctgacttgccctgcaactgatggtgactctgtctcccagagaggcagacagggaggatgtagtctgtgtcatctggatgtccggcctggcggcgtggagcagcaaggccagcggcaggagcaaggcggtcactggtaaggccatggtggctctagagtaggcgccggtcacagcttggatctgtaacggcgcagaacagaaaacgaaacaaagacgtagagttgagcaagcagggtcaggcaaagcgtggagagccggctgagtctaggtaggctccaagggagcgccggacaaaggcccggtctcgacctgagctttaaacttacctagacggcggacgcagttcaggaggcaccacaggcgggaggcggcagaacgcgactcaaccggcgtggatggcggcctcaggtagggcggcgggcgcgtgaaggagagatgcgagcccctcgaagcttcagctgtgttctggcggcaaacccgttgcgaaaaagaacgttcacggcgactactgcacttatatacggttctcccccaccctcgggaaaaaggcggagccagtacacgacatcactttcccagtttaccccgcgccaccttctctaggcacccgttcaattgccgacccctccccccaacttctcggggactgtgggcgatgtgcgctctgcccactgacgggcaccggagcggcgccctggccagtcgtctgggcggtgctacaactgggctggcggccaggatggttcttaggtaggtggggtcggcggtcaggtgtcccagagccaggggtctggagggaccttccaccctcagtccctggcaggtcggggggtgctgaggcgggcctggccctggcagcccaggggtcccggagcgaggggtctggag

SEQ ID NO: 31 - DNA, 2932 bp, Artificial Sequence
ctcgggcgggatatggaaagaggccacagcagtgagcagagacacagaggaggaaggggccctgagctggggagacccccacggggtagggcgtgggggccacgggcccacctcctccccatctcctctgtctccctgtctctgtctctctctccctcccccaccctctccccagtcctaccccctcctcacccctcctcccccagcactgcctctgtcactctcgcccacgtggatgtggaggaagagggggcgggagcaaggggcgggcaccctcccttcaacctgacctgggacagtttcccttccgctcacctccgcctgagcagtggagaaggcggcactctggtggggctgctccaggcatgcagatcccacataagatacattgatgagtttggacaaaccacaactagaatgcagtgaaaaaaatgctttatttgtgaaatttgtgatgctattgctttatttgtaaccattataagctgcaataaacaagttgtcgaggccgcggatccttcgaattcttagcgagggggcagggcctgcatgtgaagggcgtcgtaggtgtccttggtggctgtactgagaccctggtaaaggccatcgtgccccttgcccctccggcgctcgcctttcatcccaatctcactgtaggcctccgccatcttatctttctgcagttcattgtacaggccttcctgagggttcttccttctcggctttccccccatctcagggtcccggccacgtctcttgtccaaaacatcgtactcctctcttcgtcctagattgagctcgttatagagctggttctggccctgcttgtacgcgggggcgtctgcgctcctgctgaacttcactctcagttcacatcctccttcttcttcttctggaaatcggcagctacagccatcttcctcttgagtagtttgtactggtctcataaatggttgtttgaatatatacaggagtttctttctgccccgtttgcagtaaagggtgataaccagtgacaggagaaggaccccacaagtcccggccaagggcgcccagatgtagatatcacaggcgaagtccagccccctcgtgtgcactgcgccccccgccgctggccggcacgcctctgggcgcagggacaggggctgcgacgcgatggtgggcgccggtgttggtggtcgcggcgctggcgtcgtggttgaggagacggtgactgaggttccttggccccagtagtccatagcatagctaccaccgtagtaataatgtttggcacagtagtaaatggctgtgtcatcagtttgcagactgttcatttttaagaaaacttggctcttggagttgtccttgatgatggtcagtctggatttgagagctgaattatagtatgtggtttcactaccccatattactcccagccactccagaccctttcgtggaggctggcgaatccagcttacaccatagtcgggtaatgagacccctgagacagtgcatgtgacggacaggctctgtgagggcgccaccaggccaggtcctgactcctgcagtttcacctcagatccgccgccacccgacccaccaccgcccgagccaccgccacctgtgatctccagcttggtcccccctccgaacgtgtacggaagcgtattaccctgttggcaaaagtaagtggcaatatcttcttgctccaggttgctaatggtgagagaataatctgttccagacccactgccactgaaccttgatgggactcctgagtgtaatcttgatgtatggtagatcaggagtttaacagttccatctggtttctgctgataccaatttaaatatttactaatgtcctgacttgccctgcaactgatggtgactctgtctcccagagaggcagacagggaggatgtagtctgtgtcatctggatgtccggcctggcggcgtggagcagcaaggccagcggcaggagcaaggcggtcactggtaaggccatggtggctctagagtaggcgccggtcacagcttggatctgtaacggcgcagaacagaaaacgaaacaaagacgtagagttgagcaagcagggtcaggcaaagcgtggagagccggctgagtctaggtaggctccaagggagcgccggacaaaggcccggtctcgacctgagctttaaacttacctagacggcggacgcagttcaggaggcaccacaggcgggaggcggcagaacgcgactcaaccggcgtggatggcggcctcaggtagggcggcgggcgcgtgaaggagagatgcgagcccctcgaagcttcagctgtgttctggcggcaaacccgttgcgaaaaagaacgttcacggcgactactgcacttatatacggttctcccccaccctcgggaaaaaggcggagccagtacacgacatcactttcccagtttaccccgcgccaccttctctaggcacccgttcaattgccgacccctccccccaacttctcggggactgtgggcgatgtgcgctctgcccactgacgggcaccggagcggcgccctggccagtcgtctgggcggtgctacaactgggctggcggccaggatggttcttaggtaggtggggtcggcggtcaggtgtcccagagccaggggtctggagggaccttccaccctcagtccctggcaggtcggggggtgctgaggcgggcctggccctggcagcccaggggtcccggagcgaggggtctggagggacctttcactctcagtccctggcaggtcggggggtgctgtggcaggcccagccttggcccccagctctgccccttaccctgagctgtgtggctttgggcagctcgaactcctgggttcctctctgggccccaactcctcccctggcccaagtcccctctttgctcctgggcaggcaggacctctgtcccctctcagcc

SEQ ID NO: 32 - DNA, 3753 bp, Artificial Sequence
ccctgccaccgccccagcccccccgtcaggctgttgcaggcatcacacggtggaaagatctggaactgtggccatggtgtgaggccatccacaaggtggaagctttgagggggagccgattagccatggacagttgtcattcagtagggtcacctgtgccccagcgaagggggatgggccgggaaggcagaggccaggcacctgcccccagcaggggcagaggctgtgggcagccgggaggctcccagaggctccgacagaatgggagtggggttgagcccacccctcactgcagcccaggaacctgagcccagagggggccacccaccttccccaggcagggaggcccggcccccagggagatgggggggatgggggaggagaagggcctgcccccacccggcagcctcaggaggggcagctcgggcgggatatggaaagaggccacagcagtgagcagagacacagaggaggaaggggccctgagctggggagacccccacggggtagggcgtgggggccacgggcccacctcctccccatctcctctgtctccctgtctctgtctctctctccctcccccaccctctccccagtcctaccccctcctcacccctcctcccccagcactgcctctgtcactctcgcccacgtggatgtggaggaagagggggcgggagcaaggggcgggcaccctcccttcaacctgacctgggacagtttcccttccgctcacctccgcctgagcagtggagaaggcggcactctggtggggctgctccaggcatgcagatcccacataagatacattgatgagtttggacaaaccacaactagaatgcagtgaaaaaaatgctttatttgtgaaatttgtgatgctattgctttatttgtaaccattataagctgcaataaacaagttgtcgaggccgcggatccttcgaattcttagcgagggggcagggcctgcatgtgaagggcgtcgtaggtgtccttggtggctgtactgagaccctggtaaaggccatcgtgccccttgcccctccggcgctcgcctttcatcccaatctcactgtaggcctccgccatcttatctttctgcagttcattgtacaggccttcctgagggttcttccttctcggctttccccccatctcagggtcccggccacgtctcttgtccaaaacatcgtactcctctcttcgtcctagattgagctcgttatagagctggttctggccctgcttgtacgcgggggcgtctgcgctcctgctgaacttcactctcagttcacatcctccttcttcttcttctggaaatcggcagctacagccatcttcctcttgagtagtttgtactggtctcataaatggttgtttgaatatatacaggagtttctttctgccccgtttgcagtaaagggtgataaccagtgacaggagaaggaccccacaagtcccggccaagggcgcccagatgtagatatcacaggcgaagtccagccccctcgtgtgcactgcgccccccgccgctggccggcacgcctctgggcgcagggacaggggctgcgacgcgatggtgggcgccggtgttggtggtcgcggcgctggcgtcgtggttgaggagacggtgactgaggttccttggccccagtagtccatagcatagctaccaccgtagtaataatgtttggcacagtagtaaatggctgtgtcatcagtttgcagactgttcatttttaagaaaacttggctcttggagttgtccttgatgatggtcagtctggatttgagagctgaattatagtatgtggtttcactaccccatattactcccagccactccagaccctttcgtggaggctggcgaatccagcttacaccatagtcgggtaatgagacccctgagacagtgcatgtgacggacaggctctgtgagggcgccaccaggccaggtcctgactcctgcagtttcacctcagatccgccgccacccgacccaccaccgcccgagccaccgccacctgtgatctccagcttggtcccccctccgaacgtgtacggaagcgtattaccctgttggcaaaagtaagtggcaatatcttcttgctccaggttgctaatggtgagagaataatctgttccagacccactgccactgaaccttgatgggactcctgagtgtaatcttgatgtatggtagatcaggagtttaacagttccatctggtttctgctgataccaatttaaatatttactaatgtcctgacttgccctgcaactgatggtgactctgtctcccagagaggcagacagggaggatgtagtctgtgtcatctggatgtccggcctggcggcgtggagcagcaaggccagcggcaggagcaaggcggtcactggtaaggccatggtggctctagagtaggcgccggtcacagcttggatctgtaacggcgcagaacagaaaacgaaacaaagacgtagagttgagcaagcagggtcaggcaaagcgtggagagccggctgagtctaggtaggctccaagggagcgccggacaaaggcccggtctcgacctgagctttaaacttacctagacggcggacgcagttcaggaggcaccacaggcgggaggcggcagaacgcgactcaaccggcgtggatggcggcctcaggtagggcggcgggcgcgtgaaggagagatgcgagcccctcgaagcttcagctgtgttctggcggcaaacccgttgcgaaaaagaacgttcacggcgactactgcacttatatacggttctcccccaccctcgggaaaaaggcggagccagtacacgacatcactttcccagtttaccccgcgccaccttctctaggcacccgttcaattgccgacccctccccccaacttctcggggactgtgggcgatgtgcgctctgcccactgacgggcaccggagcggcgccctggccagtcgtctgggcggtgctacaactgggctggcggccaggatggttcttaggtaggtggggtcggcggtcaggtgtcccagagccaggggtctggagggaccttccaccctcagtccctggcaggtcggggggtgctgaggcgggcctggccctggcagcccaggggtcccggagcgaggggtctggagggacctttcactctcagtccctggcaggtcggggggtgctgtggcaggcccagccttggcccccagctctgccccttaccctgagctgtgtggctttgggcagctcgaactcctgggttcctctctgggccccaactcctcccctggcccaagtcccctctttgctcctgggcaggcaggacctctgtcccctctcagccggtccttggggctgcgtgtttctgtagaatgacgggtcaggctggccagaaccccaaaccttggccgtggggagtctgcgtggcggctctgccttgcccaggcatccttggtcctcactcgagttttcctaaggatgggatgagccccatgtgggactaaccttggctttacgacgtcaaagtttagatgagctggtgatatttttctcattatatccaaagtgtacctgttcgagtgaggacagttcttctgtctccaggatccctcctgggtggggattgtgcccgcctgggtctctgcccagattccagggctctccccgagccctgttcagaccatccgtgggggaggccttggcctcactctcccggatcgaggagagagggagcctcttcctgg

SEQ ID NO: 33 - DNA, 2686 bp, Artificial Sequence
tctggactccagcctgggttggggcaaagagggaaatgagatcatgtcctaaccctgatcctcttgtcccacagatatccagaaccctgaccctgccgtgtaccagctgagagactctaaatccagtgacaagtctgtctgcctattcaccgattttgattctcaaacaaatgtgtcacaaagtaaggattctgatgtgtatatcacagacaaaactgtgctagacatgaggtctatggacttcaagagcaacagtgctgtgtaagatacattgatgagtttggacaaaccacaactagaatgcagtgaaaaaaatgctttatttgtgaaatttgtgatgctattgctttatttgtaaccattataagctgcaataaacaagttgtcgaggccgcggatccttcgaattcttagcgagggggcagggcctgcatgtgaagggcgtcgtaggtgtccttggtggctgtactgagaccctggtaaaggccatcgtgccccttgcccctccggcgctcgcctttcatcccaatctcactgtaggcctccgccatcttatctttctgcagttcattgtacaggccttcctgagggttcttccttctcggctttccccccatctcagggtcccggccacgtctcttgtccaaaacatcgtactcctctcttcgtcctagattgagctcgttatagagctggttctggccctgcttgtacgcgggggcgtctgcgctcctgctgaacttcactctcagttcacatcctccttcttcttcttctggaaatcggcagctacagccatcttcctcttgagtagtttgtactggtctcataaatggttgtttgaatatatacaggagtttctttctgccccgtttgcagtaaagggtgataaccagtgacaggagaaggaccccacaagtcccggccaagggcgcccagatgtagatatcacaggcgaagtccagccccctcgtgtgcactgcgccccccgccgctggccggcacgcctctgggcgcagggacaggggctgcgacgcgatggtgggcgccggtgttggtggtcgcggcgctggcgtcgtggttgaggagacggtgactgaggttccttggccccagtagtccatagcatagctaccaccgtagtaataatgtttggcacagtagtaaatggctgtgtcatcagtttgcagactgttcatttttaagaaaacttggctcttggagttgtccttgatgatggtcagtctggatttgagagctgaattatagtatgtggtttcactaccccatattactcccagccactccagaccctttcgtggaggctggcgaatccagcttacaccatagtcgggtaatgagacccctgagacagtgcatgtgacggacaggctctgtgagggcgccaccaggccaggtcctgactcctgcagtttcacctcagatccgccgccacccgacccaccaccgcccgagccaccgccacctgtgatctccagcttggtcccccctccgaacgtgtacggaagcgtattaccctgttggcaaaagtaagtggcaatatcttcttgctccaggttgctaatggtgagagaataatctgttccagacccactgccactgaaccttgatgggactcctgagtgtaatcttgatgtatggtagatcaggagtttaacagttccatctggtttctgctgataccaatttaaatatttactaatgtcctgacttgccctgcaactgatggtgactctgtctcccagagaggcagacagggaggatgtagtctgtgtcatctggatgtccggcctggcggcgtggagcagcaaggccagcggcaggagcaaggcggtcactggtaaggccatggtggctctagagtaggcgccggtcacagcttggatctgtaacggcgcagaacagaaaacgaaacaaagacgtagagttgagcaagcagggtcaggcaaagcgtggagagccggctgagtctaggtaggctccaagggagcgccggacaaaggcccggtctcgacctgagctttaaacttacctagacggcggacgcagttcaggaggcaccacaggcgggaggcggcagaacgcgactcaaccggcgtggatggcggcctcaggtagggcggcgggcgcgtgaaggagagatgcgagcccctcgaagcttcagctgtgttctggcggcaaacccgttgcgaaaaagaacgttcacggcgactactgcacttatatacggttctcccccaccctcgggaaaaaggcggagccagtacacgacatcactttcccagtttaccccgcgccaccttctctaggcacccgttcaattgccgacccctccccccaacttctcggggactgtgggcgatgtgcgctctgcccactgacgggcaccggagcgcctggagcaacaaatctgactttgcatgtgcaaacgccttcaacaacagcattattccagaagacaccttcttccccagcccaggtaagggcagctttggtgccttcgcaggctgtttccttgcttcaggaatggccaggttctgcccagagctctggtcaatgatgtctaaaactcctctgattggtggtctcggccttatccattgccaccaaaaccctctttttactaagaaacagtgagccttgttctggcagtccagagaatgac

SEQ ID NO: 34 - DNA, 2953 bp, Artificial Sequence
ccaagattgatagcttgtgcctgtccctgagtcccagtccatcacgagcagctggtttctaagatgctatttcccgtataaagcatgagaccgtgacttgccagccccacagagccccgcccttgtccatcactggcatctggactccagcctgggttggggcaaagagggaaatgagatcatgtcctaaccctgatcctcttgtcccacagatatccagaaccctgaccctgccgtgtaccagctgagagactctaaatccagtgacaagtctgtctgcctattcaccgattttgattctcaaacaaatgtgtcacaaagtaaggattctgatgtgtatatcacagacaaaactgtgctagacatgaggtctatggacttcaagagcaacagtgctgtgtaagatacattgatgagtttggacaaaccacaactagaatgcagtgaaaaaaatgctttatttgtgaaatttgtgatgctattgctttatttgtaaccattataagctgcaataaacaagttgtcgaggccgcggatccttcgaattcttagcgagggggcagggcctgcatgtgaagggcgtcgtaggtgtccttggtggctgtactgagaccctggtaaaggccatcgtgccccttgcccctccggcgctcgcctttcatcccaatctcactgtaggcctccgccatcttatctttctgcagttcattgtacaggccttcctgagggttcttccttctcggctttccccccatctcagggtcccggccacgtctcttgtccaaaacatcgtactcctctcttcgtcctagattgagctcgttatagagctggttctggccctgcttgtacgcgggggcgtctgcgctcctgctgaacttcactctcagttcacatcctccttcttcttcttctggaaatcggcagctacagccatcttcctcttgagtagtttgtactggtctcataaatggttgtttgaatatatacaggagtttctttctgccccgtttgcagtaaagggtgataaccagtgacaggagaaggaccccacaagtcccggccaagggcgcccagatgtagatatcacaggcgaagtccagccccctcgtgtgcactgcgccccccgccgctggccggcacgcctctgggcgcagggacaggggctgcgacgcgatggtgggcgccggtgttggtggtcgcggcgctggcgtcgtggttgaggagacggtgactgaggttccttggccccagtagtccatagcatagctaccaccgtagtaataatgtttggcacagtagtaaatggctgtgtcatcagtttgcagactgttcatttttaagaaaacttggctcttggagttgtccttgatgatggtcagtctggatttgagagctgaattatagtatgtggtttcactaccccatattactcccagccactccagaccctttcgtggaggctggcgaatccagcttacaccatagtcgggtaatgagacccctgagacagtgcatgtgacggacaggctctgtgagggcgccaccaggccaggtcctgactcctgcagtttcacctcagatccgccgccacccgacccaccaccgcccgagccaccgccacctgtgatctccagcttggtcccccctccgaacgtgtacggaagcgtattaccctgttggcaaaagtaagtggcaatatcttcttgctccaggttgctaatggtgagagaataatctgttccagacccactgccactgaaccttgatgggactcctgagtgtaatcttgatgtatggtagatcaggagtttaacagttccatctggtttctgctgataccaatttaaatatttactaatgtcctgacttgccctgcaactgatggtgactctgtctcccagagaggcagacagggaggatgtagtctgtgtcatctggatgtccggcctggcggcgtggagcagcaaggccagcggcaggagcaaggcggtcactggtaaggccatggtggctctagagtaggcgccggtcacagcttggatctgtaacggcgcagaacagaaaacgaaacaaagacgtagagttgagcaagcagggtcaggcaaagcgtggagagccggctgagtctaggtaggctccaagggagcgccggacaaaggcccggtctcgacctgagctttaaacttacctagacggcggacgcagttcaggaggcaccacaggcgggaggcggcagaacgcgactcaaccggcgtggatggcggcctcaggtagggcggcgggcgcgtgaaggagagatgcgagcccctcgaagcttcagctgtgttctggcggcaaacccgttgcgaaaaagaacgttcacggcgactactgcacttatatacggttctcccccaccctcgggaaaaaggcggagccagtacacgacatcactttcccagtttaccccgcgccaccttctctaggcacccgttcaattgccgacccctccccccaacttctcggggactgtgggcgatgtgcgctctgcccactgacgggcaccggagcgcctggagcaacaaatctgactttgcatgtgcaaacgccttcaacaacagcattattccagaagacaccttcttccccagcccaggtaagggcagctttggtgccttcgcaggctgtttccttgcttcaggaatggccaggttctgcccagagctctggtcaatgatgtctaaaactcctctgattggtggtctcggccttatccattgccaccaaaaccctctttttactaagaaacagtgagccttgttctggcagtccagagaatgacacgggaaaaaagcagatgaagagaaggtggcaggagagggcacgtggcccagcctcagtctctccaactgagttcctgcctgcctgcctttgctcagactgtttgccccttactgctcttctaggcctc

SEQ ID NO: 35 - DNA, 3753 bp, Artificial Sequence
tgtgacttgctcaaggccttatatcgagtaaacggtagtgctggggcttagacgcaggtgttctgatttatagttcaaaacctctatcaatgagagagcaatctcctggtaatgtgatagatttcccaacttaatgccaacataccataaacctcccattctgctaatgcccagcctaagttggggagaccactccagattccaagatgtacagtttgctttgctgggcctttttcccatgcctgcctttactctgccagagttatattgctggggttttgaagaagatcctattaaataaaagaataagcagtattattaagtagccctgcatttcaggtttccttgagtggcaggccaggcctggccgtgaacgttcactgaaatcatggcctcttggccaagattgatagcttgtgcctgtccctgagtcccagtccatcacgagcagctggtttctaagatgctatttcccgtataaagcatgagaccgtgacttgccagccccacagagccccgcccttgtccatcactggcatctggactccagcctgggttggggcaaagagggaaatgagatcatgtcctaaccctgatcctcttgtcccacagatatccagaaccctgaccctgccgtgtaccagctgagagactctaaatccagtgacaagtctgtctgcctattcaccgattttgattctcaaacaaatgtgtcacaaagtaaggattctgatgtgtatatcacagacaaaactgtgctagacatgaggtctatggacttcaagagcaacagtgctgtgtaagatacattgatgagtttggacaaaccacaactagaatgcagtgaaaaaaatgctttatttgtgaaatttgtgatgctattgctttatttgtaaccattataagctgcaataaacaagttgtcgaggccgcggatccttcgaattcttagcgagggggcagggcctgcatgtgaagggcgtcgtaggtgtccttggtggctgtactgagaccctggtaaaggccatcgtgccccttgcccctccggcgctcgcctttcatcccaatctcactgtaggcctccgccatcttatctttctgcagttcattgtacaggccttcctgagggttcttccttctcggctttccccccatctcagggtcccggccacgtctcttgtccaaaacatcgtactcctctcttcgtcctagattgagctcgttatagagctggttctggccctgcttgtacgcgggggcgtctgcgctcctgctgaacttcactctcagttcacatcctccttcttcttcttctggaaatcggcagctacagccatcttcctcttgagtagtttgtactggtctcataaatggttgtttgaatatatacaggagtttctttctgccccgtttgcagtaaagggtgataaccagtgacaggagaaggaccccacaagtcccggccaagggcgcccagatgtagatatcacaggcgaagtccagccccctcgtgtgcactgcgccccccgccgctggccggcacgcctctgggcgcagggacaggggctgcgacgcgatggtgggcgccggtgttggtggtcgcggcgctggcgtcgtggttgaggagacggtgactgaggttccttggccccagtagtccatagcatagctaccaccgtagtaataatgtttggcacagtagtaaatggctgtgtcatcagtttgcagactgttcatttttaagaaaacttggctcttggagttgtccttgatgatggtcagtctggatttgagagctgaattatagtatgtggtttcactaccccatattactcccagccactccagaccctttcgtggaggctggcgaatccagcttacaccatagtcgggtaatgagacccctgagacagtgcatgtgacggacaggctctgtgagggcgccaccaggccaggtcctgactcctgcagtttcacctcagatccgccgccacccgacccaccaccgcccgagccaccgccacctgtgatctccagcttggtcccccctccgaacgtgtacggaagcgtattaccctgttggcaaaagtaagtggcaatatcttcttgctccaggttgctaatggtgagagaataatctgttccagacccactgccactgaaccttgatgggactcctgagtgtaatcttgatgtatggtagatcaggagtttaacagttccatctggtttctgctgataccaatttaaatatttactaatgtcctgacttgccctgcaactgatggtgactctgtctcccagagaggcagacagggaggatgtagtctgtgtcatctggatgtccggcctggcggcgtggagcagcaaggccagcggcaggagcaaggcggtcactggtaaggccatggtggctctagagtaggcgccggtcacagcttggatctgtaacggcgcagaacagaaaacgaaacaaagacgtagagttgagcaagcagggtcaggcaaagcgtggagagccggctgagtctaggtaggctccaagggagcgccggacaaaggcccggtctcgacctgagctttaaacttacctagacggcggacgcagttcaggaggcaccacaggcgggaggcggcagaacgcgactcaaccggcgtggatggcggcctcaggtagggcggcgggcgcgtgaaggagagatgcgagcccctcgaagcttcagctgtgttctggcggcaaacccgttgcgaaaaagaacgttcacggcgactactgcacttatatacggttctcccccaccctcgggaaaaaggcggagccagtacacgacatcactttcccagtttaccccgcgccaccttctctaggcacccgttcaattgccgacccctccccccaacttctcggggactgtgggcgatgtgcgctctgcccactgacgggcaccggagcgcctggagcaacaaatctgactttgcatgtgcaaacgccttcaacaacagcattattccagaagacaccttcttccccagcccaggtaagggcagctttggtgccttcgcaggctgtttccttgcttcaggaatggccaggttctgcccagagctctggtcaatgatgtctaaaactcctctgattggtggtctcggccttatccattgccaccaaaaccctctttttactaagaaacagtgagccttgttctggcagtccagagaatgacacgggaaaaaagcagatgaagagaaggtggcaggagagggcacgtggcccagcctcagtctctccaactgagttcctgcctgcctgcctttgctcagactgtttgccccttactgctcttctaggcctcattctaagccccttctccaagttgcctctccttatttctccctgtctgccaaaaaatctttcccagctcactaagtcagtctcacgcagtcactcattaacccaccaatcactgattgtgccggcacatgaatgcaccaggtgttgaagtggaggaattaaaaagtcagatgaggggtgtgcccagaggaagcaccattctagttgggggagcccatctgtcagctgggaaaagtccaaataacttcagattggaatgtgttttaactcagggttgagaaaacagctaccttcaggacaaaagtcagggaagggctctctgaagaaatgctacttgaagataccagccctaccaagggcagggagaggaccctatagaggcctgggacaggagctcaatg

SEQ ID NO: 36 - DNA, 2553 bp, Artificial Sequence
ctaagaaaaggaaactgaaaacgggaaagtccctctctctaacctggcactgcgtcgctggcttggagacaggtgacggtccctgcgggccttgtcctgattggctgggcacgcgtttaatataagtggaggcgtcgcgctggcgggcattcctgaagctgacagcattcgggccgagatgtctcgctccgtggccttagtaagatacattgatgagtttggacaaaccacaactagaatgcagtgaaaaaaatgctttatttgtgaaatttgtgatgctattgctttatttgtaaccattataagctgcaataaacaagttgtcgaggccgcggatccttcgaattcttagcgagggggcagggcctgcatgtgaagggcgtcgtaggtgtccttggtggctgtactgagaccctggtaaaggccatcgtgccccttgcccctccggcgctcgcctttcatcccaatctcactgtaggcctccgccatcttatctttctgcagttcattgtacaggccttcctgagggttcttccttctcggctttccccccatctcagggtcccggccacgtctcttgtccaaaacatcgtactcctctcttcgtcctagattgagctcgttatagagctggttctggccctgcttgtacgcgggggcgtctgcgctcctgctgaacttcactctcagttcacatcctccttcttcttcttctggaaatcggcagctacagccatcttcctcttgagtagtttgtactggtctcataaatggttgtttgaatatatacaggagtttctttctgccccgtttgcagtaaagggtgataaccagtgacaggagaaggaccccacaagtcccggccaagggcgcccagatgtagatatcacaggcgaagtccagccccctcgtgtgcactgcgccccccgccgctggccggcacgcctctgggcgcagggacaggggctgcgacgcgatggtgggcgccggtgttggtggtcgcggcgctggcgtcgtggttgaggagacggtgactgaggttccttggccccagtagtccatagcatagctaccaccgtagtaataatgtttggcacagtagtaaatggctgtgtcatcagtttgcagactgttcatttttaagaaaacttggctcttggagttgtccttgatgatggtcagtctggatttgagagctgaattatagtatgtggtttcactaccccatattactcccagccactccagaccctttcgtggaggctggcgaatccagcttacaccatagtcgggtaatgagacccctgagacagtgcatgtgacggacaggctctgtgagggcgccaccaggccaggtcctgactcctgcagtttcacctcagatccgccgccacccgacccaccaccgcccgagccaccgccacctgtgatctccagcttggtcccccctccgaacgtgtacggaagcgtattaccctgttggcaaaagtaagtggcaatatcttcttgctccaggttgctaatggtgagagaataatctgttccagacccactgccactgaaccttgatgggactcctgagtgtaatcttgatgtatggtagatcaggagtttaacagttccatctggtttctgctgataccaatttaaatatttactaatgtcctgacttgccctgcaactgatggtgactctgtctcccagagaggcagacagggaggatgtagtctgtgtcatctggatgtccggcctggcggcgtggagcagcaaggccagcggcaggagcaaggcggtcactggtaaggccatggtggctctagagtaggcgccggtcacagcttggatctgtaacggcgcagaacagaaaacgaaacaaagacgtagagttgagcaagcagggtcaggcaaagcgtggagagccggctgagtctaggtaggctccaagggagcgccggacaaaggcccggtctcgacctgagctttaaacttacctagacggcggacgcagttcaggaggcaccacaggcgggaggcggcagaacgcgactcaaccggcgtggatggcggcctcaggtagggcggcgggcgcgtgaaggagagatgcgagcccctcgaagcttcagctgtgttctggcggcaaacccgttgcgaaaaagaacgttcacggcgactactgcacttatatacggttctcccccaccctcgggaaaaaggcggagccagtacacgacatcactttcccagtttaccccgcgccaccttctctaggcacccgttcaattgccgacccctccccccaacttctcggggactgtgggcgatgtgcgctctgcccactgacgggcaccggagcctgtgctcgcgctactctctctttctggcctggaggctatccagcgtgagtctctcctaccctcccgctctggtccttcctctcccgctctgcaccctctgtggccctcgctgtgctctctcgctccgtgacttcccttctccaagttctccttggtggcccgccgtggggctagtccagggctggatctcggggaagcg

SEQ ID NO: 37 - DNA, 2953 bp, Artificial Sequence
ggcaccattagcaagtcacttagcatctctggggccagtctgcaaagcgagggggcagccttaatgtgcctccagcctgaagtcctagaatgagcgcccggtgtcccaagctggggcgcgcaccccagatcggagggcgccgatgtacagacagcaaactcacccagtctagtgcatgccttcttaaacatcacgagactctaagaaaaggaaactgaaaacgggaaagtccctctctctaacctggcactgcgtcgctggcttggagacaggtgacggtccctgcgggccttgtcctgattggctgggcacgcgtttaatataagtggaggcgtcgcgctggcgggcattcctgaagctgacagcattcgggccgagatgtctcgctccgtggccttagtaagatacattgatgagtttggacaaaccacaactagaatgcagtgaaaaaaatgctttatttgtgaaatttgtgatgctattgctttatttgtaaccattataagctgcaataaacaagttgtcgaggccgcggatccttcgaattcttagcgagggggcagggcctgcatgtgaagggcgtcgtaggtgtccttggtggctgtactgagaccctggtaaaggccatcgtgccccttgcccctccggcgctcgcctttcatcccaatctcactgtaggcctccgccatcttatctttctgcagttcattgtacaggccttcctgagggttcttccttctcggctttccccccatctcagggtcccggccacgtctcttgtccaaaacatcgtactcctctcttcgtcctagattgagctcgttatagagctggttctggccctgcttgtacgcgggggcgtctgcgctcctgctgaacttcactctcagttcacatcctccttcttcttcttctggaaatcggcagctacagccatcttcctcttgagtagtttgtactggtctcataaatggttgtttgaatatatacaggagtttctttctgccccgtttgcagtaaagggtgataaccagtgacaggagaaggaccccacaagtcccggccaagggcgcccagatgtagatatcacaggcgaagtccagccccctcgtgtgcactgcgccccccgccgctggccggcacgcctctgggcgcagggacaggggctgcgacgcgatggtgggcgccggtgttggtggtcgcggcgctggcgtcgtggttgaggagacggtgactgaggttccttggccccagtagtccatagcatagctaccaccgtagtaataatgtttggcacagtagtaaatggctgtgtcatcagtttgcagactgttcatttttaagaaaacttggctcttggagttgtccttgatgatggtcagtctggatttgagagctgaattatagtatgtggtttcactaccccatattactcccagccactccagaccctttcgtggaggctggcgaatccagcttacaccatagtcgggtaatgagacccctgagacagtgcatgtgacggacaggctctgtgagggcgccaccaggccaggtcctgactcctgcagtttcacctcagatccgccgccacccgacccaccaccgcccgagccaccgccacctgtgatctccagcttggtcccccctccgaacgtgtacggaagcgtattaccctgttggcaaaagtaagtggcaatatcttcttgctccaggttgctaatggtgagagaataatctgttccagacccactgccactgaaccttgatgggactcctgagtgtaatcttgatgtatggtagatcaggagtttaacagttccatctggtttctgctgataccaatttaaatatttactaatgtcctgacttgccctgcaactgatggtgactctgtctcccagagaggcagacagggaggatgtagtctgtgtcatctggatgtccggcctggcggcgtggagcagcaaggccagcggcaggagcaaggcggtcactggtaaggccatggtggctctagagtaggcgccggtcacagcttggatctgtaacggcgcagaacagaaaacgaaacaaagacgtagagttgagcaagcagggtcaggcaaagcgtggagagccggctgagtctaggtaggctccaagggagcgccggacaaaggcccggtctcgacctgagctttaaacttacctagacggcggacgcagttcaggaggcaccacaggcgggaggcggcagaacgcgactcaaccggcgtggatggcggcctcaggtagggcggcgggcgcgtgaaggagagatgcgagcccctcgaagcttcagctgtgttctggcggcaaacccgttgcgaaaaagaacgttcacggcgactactgcacttatatacggttctcccccaccctcgggaaaaaggcggagccagtacacgacatcactttcccagtttaccccgcgccaccttctctaggcacccgttcaattgccgacccctccccccaacttctcggggactgtgggcgatgtgcgctctgcccactgacgggcaccggagcctgtgctcgcgctactctctctttctggcctggaggctatccagcgtgagtctctcctaccctcccgctctggtccttcctctcccgctctgcaccctctgtggccctcgctgtgctctctcgctccgtgacttcccttctccaagttctccttggtggcccgccgtggggctagtccagggctggatctcggggaagcggcggggtggcctgggagtggggaagggggtgcgcacccgggacgcgcgctacttgcccctttcggcggggagcaggggagacctttggcctacggcgacgggagggtcgggacaaagtttagggcgtcgataagcgtcagagcgccgaggttgggggagggtttctcttccgctctttcgcggggcctctggctccccca

SEQ ID NO: 38 - DNA, 3753 bp, Artificial Sequence
cgctggaagctctaaagccctagcagttactgcttttactattagtggtcgtttttttctcccccccgccccccgacaaatcaacagaacaaagaaaattacctaaacagcaaggacatagggaggaacttcttggcacagaactttccaaacactttttcctgaagggatacaagaagcaagaaaggtactctttcactaggaccttctctgagctgtcctcaggatgcttttgggactatttttcttacccagagaatggagaaaccctgcagggaattcccaagctgtagttataaacagaagttctccttctgctaggtagcattcaaagatcttaatcttctgggtttccgttttctcgaatgaaaaatgcaggtccgagcagttaactggctggggcaccattagcaagtcacttagcatctctggggccagtctgcaaagcgagggggcagccttaatgtgcctccagcctgaagtcctagaatgagcgcccggtgtcccaagctggggcgcgcaccccagatcggagggcgccgatgtacagacagcaaactcacccagtctagtgcatgccttcttaaacatcacgagactctaagaaaaggaaactgaaaacgggaaagtccctctctctaacctggcactgcgtcgctggcttggagacaggtgacggtccctgcgggccttgtcctgattggctgggcacgcgtttaatataagtggaggcgtcgcgctggcgggcattcctgaagctgacagcattcgggccgagatgtctcgctccgtggccttagtaagatacattgatgagtttggacaaaccacaactagaatgcagtgaaaaaaatgctttatttgtgaaatttgtgatgctattgctttatttgtaaccattataagctgcaataaacaagttgtcgaggccgcggatccttcgaattcttagcgagggggcagggcctgcatgtgaagggcgtcgtaggtgtccttggtggctgtactgagaccctggtaaaggccatcgtgccccttgcccctccggcgctcgcctttcatcccaatctcactgtaggcctccgccatcttatctttctgcagttcattgtacaggccttcctgagggttcttccttctcggctttccccccatctcagggtcccggccacgtctcttgtccaaaacatcgtactcctctcttcgtcctagattgagctcgttatagagctggttctggccctgcttgtacgcgggggcgtctgcgctcctgctgaacttcactctcagttcacatcctccttcttcttcttctggaaatcggcagctacagccatcttcctcttgagtagtttgtactggtctcataaatggttgtttgaatatatacaggagtttctttctgccccgtttgcagtaaagggtgataaccagtgacaggagaaggaccccacaagtcccggccaagggcgcccagatgtagatatcacaggcgaagtccagccccctcgtgtgcactgcgccccccgccgctggccggcacgcctctgggcgcagggacaggggctgcgacgcgatggtgggcgccggtgttggtggtcgcggcgctggcgtcgtggttgaggagacggtgactgaggttccttggccccagtagtccatagcatagctaccaccgtagtaataatgtttggcacagtagtaaatggctgtgtcatcagtttgcagactgttcatttttaagaaaacttggctcttggagttgtccttgatgatggtcagtctggatttgagagctgaattatagtatgtggtttcactaccccatattactcccagccactccagaccctttcgtggaggctggcgaatccagcttacaccatagtcgggtaatgagacccctgagacagtgcatgtgacggacaggctctgtgagggcgccaccaggccaggtcctgactcctgcagtttcacctcagatccgccgccacccgacccaccaccgcccgagccaccgccacctgtgatctccagcttggtcccccctccgaacgtgtacggaagcgtattaccctgttggcaaaagtaagtggcaatatcttcttgctccaggttgctaatggtgagagaataatctgttccagacccactgccactgaaccttgatgggactcctgagtgtaatcttgatgtatggtagatcaggagtttaacagttccatctggtttctgctgataccaatttaaatatttactaatgtcctgacttgccctgcaactgatggtgactctgtctcccagagaggcagacagggaggatgtagtctgtgtcatctggatgtccggcctggcggcgtggagcagcaaggccagcggcaggagcaaggcggtcactggtaaggccatggtggctctagagtaggcgccggtcacagcttggatctgtaacggcgcagaacagaaaacgaaacaaagacgtagagttgagcaagcagggtcaggcaaagcgtggagagccggctgagtctaggtaggctccaagggagcgccggacaaaggcccggtctcgacctgagctttaaacttacctagacggcggacgcagttcaggaggcaccacaggcgggaggcggcagaacgcgactcaaccggcgtggatggcggcctcaggtagggcggcgggcgcgtgaaggagagatgcgagcccctcgaagcttcagctgtgttctggcggcaaacccgttgcgaaaaagaacgttcacggcgactactgcacttatatacggttctcccccaccctcgggaaaaaggcggagccagtacacgacatcactttcccagtttaccccgcgccaccttctctaggcacccgttcaattgccgacccctccccccaacttctcggggactgtgggcgatgtgcgctctgcccactgacgggcaccggagcctgtgctcgcgctactctctctttctggcctggaggctatccagcgtgagtctctcctaccctcccgctctggtccttcctctcccgctctgcaccctctgtggccctcgctgtgctctctcgctccgtgacttcccttctccaagttctccttggtggcccgccgtggggctagtccagggctggatctcggggaagcggcggggtggcctgggagtggggaagggggtgcgcacccgggacgcgcgctacttgcccctttcggcggggagcaggggagacctttggcctacggcgacgggagggtcgggacaaagtttagggcgtcgataagcgtcagagcgccgaggttgggggagggtttctcttccgctctttcgcggggcctctggctcccccagcgcagctggagtgggggacgggtaggctcgtcccaaaggcgcggcgctgaggtttgtgaacgcgtggaggggcgcttggggtctgggggaggcgtcgcccgggtaagcctgtctgctgcggctctgcttcccttagactggagagctgtggacttcgtctaggcgcccgctaagttcgcatgtcctagcacctctgggtctatgtggggccacaccgtggggaggaaacagcacgcgacgtttgtagaatgcttggctgtgatacaaagcggtttcgaataattaacttatttgttcccatcacatgtcacttttaaaaaattataagaactacccgttattgacatctttctgtgtgccaaggactttatgtgctttgcgtcatttaattttgaaaac

SEQ ID NO: 39 - DNA, 1577 bp, Artificial Sequence
cgactggccagggcgcctgtgggtgggcggaactgggcggagttaggggcgggatgggcggagttaggggcgggatagctagagccagacatgataagatacattgatgagtttggacaaaccacaactagaatgcagtgaaaaaaatgctttatttgtgaaatttgtgatgctattgctttatttgtaaccattataagctgcaataaacaagttgtcgaggccgcggatccttcgaattctcacttgtacagctcgtccatgccgagagtgatcccggcggcggtcacgaactccagcaggaccatgtgatcgcgcttctcgttggggtctttgctcagcttggactgggtgctcaggtagtggttgtcgggcagcagcacggggccgtcgccgatgggggtgttctgctggtagtggtcggcgagctgcacgccgccgtcctcgatgttgtggcggatcttgaagttggccttgatgccgttcttctgcttgtcggcggtgatatagacgttgtcgctgaagtagttgtactccagcttgtgccccaggatgttgccgtcctccttgaagtcgatgcccttcagctcgatgcggttcaccagggtgtcgccctcgaacttcacctcggcgcgggtcttgtagttgccgtcgtccttgaagaagatggtgcgctcctggacgtagccttcgggcatggcggacttgaagaagtcgtgctgcttcatgtggtcggggtagcgggcgaagcactgcacgccccagctcagggtggtcacgagggtgggccagggcacgggcagcttgccggtggtgcagatgaacttcagggtcagcttgccgtaggtggcatcgccctcgccctcgccggacacgctgaacttgtggccgtttacgtcgccgtccagctcgaccaggatgggcaccaccccggtgaacagctcctcgcccttgctcaccatggtggctctagagtaggcgccggtcacagcttggatctgtaacggcgcagaacagaaaacgaaacaaagacgtagagttgagcaagcagggtcaggcaaagcgtggagagccggctgagtctaggtaggctccaagggagcgccggacaaaggcccggtctcgacctgagctttaaacttacctagacggcggacgcagttcaggaggcaccacaggcgggaggcggcagaacgcgactcaaccggcgtggatggcggcctcaggtagggcggcgggcgcgtgaaggagagatgcgagcccctcgaagcttcagctgtgttctggcggcaaacccgttgcgaaaaagaacgttcacggcgactactgcacttatatacggttctcccccaccctcgggaaaaaggcggagccagtacacgacatcactttcccagtttaccccgcgccaccttctctaggcacccgttcaattgccgacccctccccccaacttctcggggactgtgggcgatgtgcgctctgcccactgacgggcaccggagcgatcgcagatccactagtatcgataaaattttgaatttttgtaatttgcgactggccagggcgcctgtggg

SEQ ID NO: 40 - DNA, 1458 bp, Artificial Sequence
cgactggccagggcgcctgtgggtaagatacattgatgagtttggacaaaccacaactagaatgcagtgaaaaaaatgctttatttgtgaaatttgtgatgctattgctttatttgtaaccattataagctgcaataaacaagttgtcgaggccgcggatccttcgaattctcacttgtacagctcgtccatgccgagagtgatcccggcggcggtcacgaactccagcaggaccatgtgatcgcgcttctcgttggggtctttgctcagcttggactgggtgctcaggtagtggttgtcgggcagcagcacggggccgtcgccgatgggggtgttctgctggtagtggtcggcgagctgcacgccgccgtcctcgatgttgtggcggatcttgaagttggccttgatgccgttcttctgcttgtcggcggtgatatagacgttgtcgctgaagtagttgtactccagcttgtgccccaggatgttgccgtcctccttgaagtcgatgcccttcagctcgatgcggttcaccagggtgtcgccctcgaacttcacctcggcgcgggtcttgtagttgccgtcgtccttgaagaagatggtgcgctcctggacgtagccttcgggcatggcggacttgaagaagtcgtgctgcttcatgtggtcggggtagcgggcgaagcactgcacgccccagctcagggtggtcacgagggtgggccagggcacgggcagcttgccggtggtgcagatgaacttcagggtcagcttgccgtaggtggcatcgccctcgccctcgccggacacgctgaacttgtggccgtttacgtcgccgtccagctcgaccaggatgggcaccaccccggtgaacagctcctcgcccttgctcaccatggtggctctagagtaggcgccggtcacagcttggatctgtaacggcgcagaacagaaaacgaaacaaagacgtagagttgagcaagcagggtcaggcaaagcgtggagagccggctgagtctaggtaggctccaagggagcgccggacaaaggcccggtctcgacctgagctttaaacttacctagacggcggacgcagttcaggaggcaccacaggcgggaggcggcagaacgcgactcaaccggcgtggatggcggcctcaggtagggcggcgggcgcgtgaaggagagatgcgagcccctcgaagcttcagctgtgttctggcggcaaacccgttgcgaaaaagaacgttcacggcgactactgcacttatatacggttctcccccaccctcgggaaaaaggcggagccagtacacgacatcactttcccagtttaccccgcgccaccttctctaggcacccgttcaattgccgacccctccccccaacttctcggggactgtgggcgatgtgcgctctgcccactgacgggcaccggagccgactggccagggcgcctgtggg

SEQ ID NO: 41 - DNA, 1498 bp, Artificial Sequence
cgactggccagggcgcctgtgggccaggcatgcagatcccacataagatacattgatgagtttggacaaaccacaactagaatgcagtgaaaaaaatgctttatttgtgaaatttgtgatgctattgctttatttgtaaccattataagctgcaataaacaagttgtcgaggccgcggatccttcgaattctcacttgtacagctcgtccatgccgagagtgatcccggcggcggtcacgaactccagcaggaccatgtgatcgcgcttctcgttggggtctttgctcagcttggactgggtgctcaggtagtggttgtcgggcagcagcacggggccgtcgccgatgggggtgttctgctggtagtggtcggcgagctgcacgccgccgtcctcgatgttgtggcggatcttgaagttggccttgatgccgttcttctgcttgtcggcggtgatatagacgttgtcgctgaagtagttgtactccagcttgtgccccaggatgttgccgtcctccttgaagtcgatgcccttcagctcgatgcggttcaccagggtgtcgccctcgaacttcacctcggcgcgggtcttgtagttgccgtcgtccttgaagaagatggtgcgctcctggacgtagccttcgggcatggcggacttgaagaagtcgtgctgcttcatgtggtcggggtagcgggcgaagcactgcacgccccagctcagggtggtcacgagggtgggccagggcacgggcagcttgccggtggtgcagatgaacttcagggtcagcttgccgtaggtggcatcgccctcgccctcgccggacacgctgaacttgtggccgtttacgtcgccgtccagctcgaccaggatgggcaccaccccggtgaacagctcctcgcccttgctcaccatggtggctctagagtaggcgccggtcacagcttggatctgtaacggcgcagaacagaaaacgaaacaaagacgtagagttgagcaagcagggtcaggcaaagcgtggagagccggctgagtctaggtaggctccaagggagcgccggacaaaggcccggtctcgacctgagctttaaacttacctagacggcggacgcagttcaggaggcaccacaggcgggaggcggcagaacgcgactcaaccggcgtggatggcggcctcaggtagggcggcgggcgcgtgaaggagagatgcgagcccctcgaagcttcagctgtgttctggcggcaaacccgttgcgaaaaagaacgttcacggcgactactgcacttatatacggttctcccccaccctcgggaaaaaggcggagccagtacacgacatcactttcccagtttaccccgcgccaccttctctaggcacccgttcaattgccgacccctccccccaacttctcggggactgtgggcgatgtgcgctctgcccactgacgggcaccggagcggcgccctggccagtcgtctcccacaggcgccctggccagtcg

SEQ ID NO: 42 - DNA, 1577 bp, Artificial Sequence
ccagcccagttgtagcaccgccctgggcggaactgggcggagttaggggcgggatgggcggagttaggggcgggatagctagagccagacatgataagatacattgatgagtttggacaaaccacaactagaatgcagtgaaaaaaatgctttatttgtgaaatttgtgatgctattgctttatttgtaaccattataagctgcaataaacaagttgtcgaggccgcggatccttcgaattctcacttgtacagctcgtccatgccgagagtgatcccggcggcggtcacgaactccagcaggaccatgtgatcgcgcttctcgttggggtctttgctcagcttggactgggtgctcaggtagtggttgtcgggcagcagcacggggccgtcgccgatgggggtgttctgctggtagtggtcggcgagctgcacgccgccgtcctcgatgttgtggcggatcttgaagttggccttgatgccgttcttctgcttgtcggcggtgatatagacgttgtcgctgaagtagttgtactccagcttgtgccccaggatgttgccgtcctccttgaagtcgatgcccttcagctcgatgcggttcaccagggtgtcgccctcgaacttcacctcggcgcgggtcttgtagttgccgtcgtccttgaagaagatggtgcgctcctggacgtagccttcgggcatggcggacttgaagaagtcgtgctgcttcatgtggtcggggtagcgggcgaagcactgcacgccccagctcagggtggtcacgagggtgggccagggcacgggcagcttgccggtggtgcagatgaacttcagggtcagcttgccgtaggtggcatcgccctcgccctcgccggacacgctgaacttgtggccgtttacgtcgccgtccagctcgaccaggatgggcaccaccccggtgaacagctcctcgcccttgctcaccatggtggctctagagtaggcgccggtcacagcttggatctgtaacggcgcagaacagaaaacgaaacaaagacgtagagttgagcaagcagggtcaggcaaagcgtggagagccggctgagtctaggtaggctccaagggagcgccggacaaaggcccggtctcgacctgagctttaaacttacctagacggcggacgcagttcaggaggcaccacaggcgggaggcggcagaacgcgactcaaccggcgtggatggcggcctcaggtagggcggcgggcgcgtgaaggagagatgcgagcccctcgaagcttcagctgtgttctggcggcaaacccgttgcgaaaaagaacgttcacggcgactactgcacttatatacggttctcccccaccctcgggaaaaaggcggagccagtacacgacatcactttcccagtttaccccgcgccaccttctctaggcacccgttcaattgccgacccctccccccaacttctcggggactgtgggcgatgtgcgctctgcccactgacgggcaccggagcgatcgcagatccactagtatcgataaaattttgaatttttgtaatttgccagcccagttgtagcaccgccc

SEQ ID NO: 43 - DNA, 1458 bp, Artificial Sequence
ccagcccagttgtagcaccgccctaagatacattgatgagtttggacaaaccacaactagaatgcagtgaaaaaaatgctttatttgtgaaatttgtgatgctattgctttatttgtaaccattataagctgcaataaacaagttgtcgaggccgcggatccttcgaattctcacttgtacagctcgtccatgccgagagtgatcccggcggcggtcacgaactccagcaggaccatgtgatcgcgcttctcgttggggtctttgctcagcttggactgggtgctcaggtagtggttgtcgggcagcagcacggggccgtcgccgatgggggtgttctgctggtagtggtcggcgagctgcacgccgccgtcctcgatgttgtggcggatcttgaagttggccttgatgccgttcttctgcttgtcggcggtgatatagacgttgtcgctgaagtagttgtactccagcttgtgccccaggatgttgccgtcctccttgaagtcgatgcccttcagctcgatgcggttcaccagggtgtcgccctcgaacttcacctcggcgcgggtcttgtagttgccgtcgtccttgaagaagatggtgcgctcctggacgtagccttcgggcatggcggacttgaagaagtcgtgctgcttcatgtggtcggggtagcgggcgaagcactgcacgccccagctcagggtggtcacgagggtgggccagggcacgggcagcttgccggtggtgcagatgaacttcagggtcagcttgccgtaggtggcatcgccctcgccctcgccggacacgctgaacttgtggccgtttacgtcgccgtccagctcgaccaggatgggcaccaccccggtgaacagctcctcgcccttgctcaccatggtggctctagagtaggcgccggtcacagcttggatctgtaacggcgcagaacagaaaacgaaacaaagacgtagagttgagcaagcagggtcaggcaaagcgtggagagccggctgagtctaggtaggctccaagggagcgccggacaaaggcccggtctcgacctgagctttaaacttacctagacggcggacgcagttcaggaggcaccacaggcgggaggcggcagaacgcgactcaaccggcgtggatggcggcctcaggtagggcggcgggcgcgtgaaggagagatgcgagcccctcgaagcttcagctgtgttctggcggcaaacccgttgcgaaaaagaacgttcacggcgactactgcacttatatacggttctcccccaccctcgggaaaaaggcggagccagtacacgacatcactttcccagtttaccccgcgccaccttctctaggcacccgttcaattgccgacccctccccccaacttctcggggactgtgggcgatgtgcgctctgcccactgacgggcaccggagcccagcccagttgtagcaccgccc

SEQ ID NO: 44 - DNA, 1498 bp, Artificial Sequence
  44
ccagcccagttgtagcaccgccctctgggcggtgctacaactgtaagatacattgatgagtttggacaaaccacaactagaatgcagtgaaaaaaatgctttatttgtgaaatttgtgatgctattgctttatttgtaaccattataagctgcaataaacaagttgtcgaggccgcggatccttcgaattctcacttgtacagctcgtccatgccgagagtgatcccggcggcggtcacgaactccagcaggaccatgtgatcgcgcttctcgttggggtctttgctcagcttggactgggtgctcaggtagtggttgtcgggcagcagcacggggccgtcgccgatgggggtgttctgctggtagtggtcggcgagctgcacgccgccgtcctcgatgttgtggcggatcttgaagttggccttgatgccgttcttctgcttgtcggcggtgatatagacgttgtcgctgaagtagttgtactccagcttgtgccccaggatgttgccgtcctccttgaagtcgatgcccttcagctcgatgcggttcaccagggtgtcgccctcgaacttcacctcggcgcgggtcttgtagttgccgtcgtccttgaagaagatggtgcgctcctggacgtagccttcgggcatggcggacttgaagaagtcgtgctgcttcatgtggtcggggtagcgggcgaagcactgcacgccccagctcagggtggtcacgagggtgggccagggcacgggcagcttgccggtggtgcagatgaacttcagggtcagcttgccgtaggtggcatcgccctcgccctcgccggacacgctgaacttgtggccgtttacgtcgccgtccagctcgaccaggatgggcaccaccccggtgaacagctcctcgcccttgctcaccatggtggctctagagtaggcgccggtcacagcttggatctgtaacggcgcagaacagaaaacgaaacaaagacgtagagttgagcaagcagggtcaggcaaagcgtggagagccggctgagtctaggtaggctccaagggagcgccggacaaaggcccggtctcgacctgagctttaaacttacctagacggcggacgcagttcaggaggcaccacaggcgggaggcggcagaacgcgactcaaccggcgtggatggcggcctcaggtagggcggcgggcgcgtgaaggagagatgcgagcccctcgaagcttcagctgtgttctggcggcaaacccgttgcgaaaaagaacgttcacggcgactactgcacttatatacggttctcccccaccctcgggaaaaaggcggagccagtacacgacatcactttcccagtttaccccgcgccaccttctctaggcacccgttcaattgccgacccctccccccaacttctcggggactgtgggcgatgtgcgctctgcccactgacgggcaccggagcggctggcggccaggatggttgggcggtgctacaactgggctgg